European Patent Application EP 4 162 950 A1, published April 12, 2023. Title: NUCLEIC ACID VACCINES FOR CORONAVIRUS. Applicant: SUZHOU ABOGEN BIOSCIENCES CO., LTD. The sequence listing filed with the application follows.

SEQUENCE LISTING (99 sequences)

SEQ ID NO: 1 - DNA, 29903 bp, Severe acute respiratory syndrome coronavirus 2 (SARS-CoV-2)
  misc_feature 1..29903: note = Severe acute respiratory syndrome coronavirus 2 isolateWuhan-Hu-1, complete genome
  source 1..29903: mol_type = genomic DNA
attaaaggtttataccttcccaggtaacaaaccaaccaactttcgatctcttgtagatctgttctctaaacgaactttaaaatctgtgtggctgtcactcggctgcatgcttagtgcactcacgcagtataattaataactaattactgtcgttgacaggacacgagtaactcgtctatcttctgcaggctgcttacggtttcgtccgtgttgcagccgatcatcagcacatctaggtttcgtccgggtgtgaccgaaaggtaagatggagagccttgtccctggtttcaacgagaaaacacacgtccaactcagtttgcctgttttacaggttcgcgacgtgctcgtacgtggctttggagactccgtggaggaggtcttatcagaggcacgtcaacatcttaaagatggcacttgtggcttagtagaagttgaaaaaggcgttttgcctcaacttgaacagccctatgtgttcatcaaacgttcggatgctcgaactgcacctcatggtcatgttatggttgagctggtagcagaactcgaaggcattcagtacggtcgtagtggtgagacacttggtgtccttgtccctcatgtgggcgaaataccagtggcttaccgcaaggttcttcttcgtaagaacggtaataaaggagctggtggccatagttacggcgccgatctaaagtcatttgacttaggcgacgagcttggcactgatccttatgaagattttcaagaaaactggaacactaaacatagcagtggtgttacccgtgaactcatgcgtgagcttaacggaggggcatacactcgctatgtcgataacaacttctgtggccctgatggctaccctcttgagtgcattaaagaccttctagcacgtgctggtaaagcttcatgcactttgtccgaacaactggactttattgacactaagaggggtgtatactgctgccgtgaacatgagcatgaaattgcttggtacacggaacgttctgaaaagagctatgaattgcagacaccttttgaaattaaattggcaaagaaatttgacaccttcaatggggaatgtccaaattttgtatttcccttaaattccataatcaagactattcaaccaagggttgaaaagaaaaagcttgatggctttatgggtagaattcgatctgtctatccagttgcgtcaccaaatgaatgcaaccaaatgtgcctttcaactctcatgaagtgtgatcattgtggtgaaacttcatggcagacgggcgattttgttaaagccacttgcgaattttgtggcactgagaatttgactaaagaaggtgccactacttgtggttacttaccccaaaatgctgttgttaaaatttattgtccagcatgtcacaattcagaagtaggacctgagcatagtcttgccgaataccataatgaatctggcttgaaaaccattcttcgtaagggtggtcgcactattgcctttggaggctgtgtgttctcttatgttggttgccataacaagtgtgcctattgggttccacgtgctagcgctaacataggttgtaaccatacaggtgttgttggagaaggttccgaaggtcttaatgacaaccttcttgaaatactccaaaaagagaaagtcaacatcaatattgttggtgactttaaacttaatgaagagatcgccattattttggcatctttttctgcttccacaagtgcttttgtggaaactgtgaaaggtttggattataaagcattcaaacaaattgttgaatcctgtggtaattttaaagttacaaaaggaaaagctaaaaaaggtgcctggaatattggtgaacagaaatcaatactgagtcctctttatgcatttgcatcagaggctgctcgtgttgtacgatcaattttctcccgcactcttgaaactgctcaaaattctgtgcgtgttttacagaaggccgctataacaatactagatggaatttcacagtattcactgagactcattgatgctatgatgttcacatctgatttggctactaacaatctagttgtaatggcctacattacaggtggtgttgttcagttgacttcgcagtggctaactaacatctttggcactgtttatgaaaaactcaaacccgtccttgattggcttgaagagaagtttaaggaaggtgtagagtttcttagagacggttgggaaattgttaaatttatctcaacctgtgcttgtgaaattgtcggtggacaaattgtcacctgtgcaaaggaaattaaggagagtgttcagacattctttaagcttgtaaataaatttttggctttgtgtgctgactctatcattattggtggagctaaacttaaagccttgaatttaggtgaaacatttgtcacgcactcaaagggattgtacagaaagtgtgttaaatccagagaagaaactggcctactcatgcctctaaaagccccaaaagaaattatcttcttagagggagaaacacttcccacagaagtgttaacagaggaagttgtcttgaaaactggtgatttacaaccattagaacaacctactagtgaagctgttgaagctccattggttggtacaccagtttgtattaacgggcttatgttgctcgaaatcaaagacacagaaaagtactgtgcccttgcacctaatatgatggtaacaaacaataccttcacactcaaaggcggtgcaccaacaaaggttacttttggtgatgacactgtgatagaagtgcaaggttacaagagtgtgaatatcacttttgaacttgatgaaaggattgataaagtacttaatgagaagtgctctgcctatacagttgaactcggtacagaagtaaatgagttcgcctgtgttgtggcagatgctgtcataaaaactttgcaaccagtatctgaattacttacaccactgggcattgatttagatgagtggagtatggctacatactacttatttgatgagtctggtgagtttaaattggcttcacatatgtattgttctttctaccctccagatgaggatgaagaagaaggtgattgtgaagaagaagagtttgagccatcaactcaatatgagtatggtactgaagatgattaccaaggtaaacctttggaatttggtgccacttctgctgctcttcaacctgaagaagagcaagaagaagattggttagatgatgatagtcaacaaactgttggtcaacaagacggcagtgaggacaatcagacaactactattcaaacaattgttgaggttcaacctcaattagagatggaacttacaccagttgttcagactattgaagtgaatagttttagtggttatttaaaacttactgacaatgtatacattaaaaatgcagacattgtggaagaagctaaaaaggtaaaaccaacagtggttgttaatgcagccaatgtttaccttaaacatggaggaggtgttgcaggagccttaaataaggctactaacaatgccatgcaagttgaatctgatgattacatagctactaatggaccacttaaagtgggtggtagttgtgttttaagcggacacaatcttgctaaacactgtcttcatgttgtcggcccaaatgttaacaaaggtgaagacattcaacttcttaagagtgcttatgaaaattttaatcagcacgaagttctacttgcaccattattatcagctggtatttttggtgctgaccctatacattctttaagagtttgtgtagatactgttcgcacaaatgtctacttagctgtctttgataaaaatctctatgacaaacttgtttcaagctttttggaaatgaagagtgaaaagcaagttgaacaaaagatcgctgagattcctaaagaggaagttaagccatttataactgaaagtaaaccttcagttgaacagagaaaacaagatgataagaaaatcaaagcttgtgttgaagaagttacaacaactctggaagaaactaagttcctcacagaaaacttgttactttatattgacattaatggcaatcttcatccagattctgccactcttgttagtgacattgacatcactttcttaaagaaagatgctccatatatagtgggtgatgttgttcaagagggtgttttaactgctgtggttatacctactaaaaaggctggtggcactactgaaatgctagcgaaagctttgagaaaagtgccaacagacaattatataaccacttacccgggtcagggtttaaatggttacactgtagaggaggcaaagacagtgcttaaaaagtgtaaaagtgccttttacattctaccatctattatctctaatgagaagcaagaaattcttggaactgtttcttggaatttgcgagaaatgcttgcacatgcagaagaaacacgcaaattaatgcctgtctgtgtggaaactaaagccatagtttcaactatacagcgtaaatataagggtattaaaatacaagagggtgtggttgattatggtgctagattttacttttacaccagtaaaacaactgtagcgtcacttatcaacacacttaacgatctaaatgaaactcttgttacaatgccacttggctatgtaacacatggcttaaatttggaagaagctgctcggtatatgagatctctcaaagtgccagctacagtttctgtttcttcacctgatgctgttacagcgtataatggttatcttacttcttcttctaaaacacctgaagaacattttattgaaaccatctcacttgctggttcctataaagattggtcctattctggacaatctacacaactaggtatagaatttcttaagagaggtgataaaagtgtatattacactagtaatcctaccacattccacctagatggtgaagttatcacctttgacaatcttaagacacttctttctttgagagaagtgaggactattaaggtgtttacaacagtagacaacattaacctccacacgcaagttgtggacatgtcaatgacatatggacaacagtttggtccaacttatttggatggagctgatgttactaaaataaaacctcataattcacatgaaggtaaaacattttatgttttacctaatgatgacactctacgtgttgaggcttttgagtactaccacacaactgatcctagttttctgggtaggtacatgtcagcattaaatcacactaaaaagtggaaatacccacaagttaatggtttaacttctattaaatgggcagataacaactgttatcttgccactgcattgttaacactccaacaaatagagttgaagtttaatccacctgctctacaagatgcttattacagagcaagggctggtgaagctgctaacttttgtgcacttatcttagcctactgtaataagacagtaggtgagttaggtgatgttagagaaacaatgagttacttgtttcaacatgccaatttagattcttgcaaaagagtcttgaacgtggtgtgtaaaacttgtggacaacagcagacaacccttaagggtgtagaagctgttatgtacatgggcacactttcttatgaacaatttaagaaaggtgttcagataccttgtacgtgtggtaaacaagctacaaaatatctagtacaacaggagtcaccttttgttatgatgtcagcaccacctgctcagtatgaacttaagcatggtacatttacttgtgctagtgagtacactggtaattaccagtgtggtcactataaacatataacttctaaagaaactttgtattgcatagacggtgctttacttacaaagtcctcagaatacaaaggtcctattacggatgttttctacaaagaaaacagttacacaacaaccataaaaccagttacttataaattggatggtgttgtttgtacagaaattgaccctaagttggacaattattataagaaagacaattcttatttcacagagcaaccaattgatcttgtaccaaaccaaccatatccaaacgcaagcttcgataattttaagtttgtatgtgataatatcaaatttgctgatgatttaaaccagttaactggttataagaaacctgcttcaagagagcttaaagttacatttttccctgacttaaatggtgatgtggtggctattgattataaacactacacaccctcttttaagaaaggagctaaattgttacataaacctattgtttggcatgttaacaatgcaactaataaagccacgtataaaccaaatacctggtgtatacgttgtctttggagcacaaaaccagttgaaacatcaaattcgtttgatgtactgaagtcagaggacgcgcagggaatggataatcttgcctgcgaagatctaaaaccagtctctgaagaagtagtggaaaatcctaccatacagaaagacgttcttgagtgtaatgtgaaaactaccgaagttgtaggagacattatacttaaaccagcaaataatagtttaaaaattacagaagaggttggccacacagatctaatggctgcttatgtagacaattctagtcttactattaagaaacctaatgaattatctagagtattaggtttgaaaacccttgctactcatggtttagctgctgttaatagtgtcccttgggatactatagctaattatgctaagccttttcttaacaaagttgttagtacaactactaacatagttacacggtgtttaaaccgtgtttgtactaattatatgccttatttctttactttattgctacaattgtgtacttttactagaagtacaaattctagaattaaagcatctatgccgactactatagcaaagaatactgttaagagtgtcggtaaattttgtctagaggcttcatttaattatttgaagtcacctaatttttctaaactgataaatattataatttggtttttactattaagtgtttgcctaggttctttaatctactcaaccgctgctttaggtgttttaatgtctaatttaggcatgccttcttactgtactggttacagagaaggctatttgaactctactaatgtcactattgcaacctactgtactggttctataccttgtagtgtttgtcttagtggtttagattctttagacacctatccttctttagaaactatacaaattaccatttcatcttttaaatgggatttaactgcttttggcttagttgcagagtggtttttggcatatattcttttcactaggtttttctatgtacttggattggctgcaatcatgcaattgtttttcagctattttgcagtacattttattagtaattcttggcttatgtggttaataattaatcttgtacaaatggccccgatttcagctatggttagaatgtacatcttctttgcatcattttattatgtatggaaaagttatgtgcatgttgtagacggttgtaattcatcaacttgtatgatgtgttacaaacgtaatagagcaacaagagtcgaatgtacaactattgttaatggtgttagaaggtccttttatgtctatgctaatggaggtaaaggcttttgcaaactacacaattggaattgtgttaattgtgatacattctgtgctggtagtacatttattagtgatgaagttgcgagagacttgtcactacagtttaaaagaccaataaatcctactgaccagtcttcttacatcgttgatagtgttacagtgaagaatggttccatccatctttactttgataaagctggtcaaaagacttatgaaagacattctctctctcattttgttaacttagacaacctgagagctaataacactaaaggttcattgcctattaatgttatagtttttgatggtaaatcaaaatgtgaagaatcatctgcaaaatcagcgtctgtttactacagtcagcttatgtgtcaacctatactgttactagatcaggcattagtgtctgatgttggtgatagtgcggaagttgcagttaaaatgtttgatgcttacgttaatacgttttcatcaacttttaacgtaccaatggaaaaactcaaaacactagttgcaactgcagaagctgaacttgcaaagaatgtgtccttagacaatgtcttatctacttttatttcagcagctcggcaagggtttgttgattcagatgtagaaactaaagatgttgttgaatgtcttaaattgtcacatcaatctgacatagaagttactggcgatagttgtaataactatatgctcacctataacaaagttgaaaacatgacaccccgtgaccttggtgcttgtattgactgtagtgcgcgtcatattaatgcgcaggtagcaaaaagtcacaacattgctttgatatggaacgttaaagatttcatgtcattgtctgaacaactacgaaaacaaatacgtagtgctgctaaaaagaataacttaccttttaagttgacatgtgcaactactagacaagttgttaatgttgtaacaacaaagatagcacttaagggtggtaaaattgttaataattggttgaagcagttaattaaagttacacttgtgttcctttttgttgctgctattttctatttaataacacctgttcatgtcatgtctaaacatactgacttttcaagtgaaatcataggatacaaggctattgatggtggtgtcactcgtgacatagcatctacagatacttgttttgctaacaaacatgctgattttgacacatggtttagccagcgtggtggtagttatactaatgacaaagcttgcccattgattgctgcagtcataacaagagaagtgggttttgtcgtgcctggtttgcctggcacgatattacgcacaactaatggtgactttttgcatttcttacctagagtttttagtgcagttggtaacatctgttacacaccatcaaaacttatagagtacactgactttgcaacatcagcttgtgttttggctgctgaatgtacaatttttaaagatgcttctggtaagccagtaccatattgttatgataccaatgtactagaaggttctgttgcttatgaaagtttacgccctgacacacgttatgtgctcatggatggctctattattcaatttcctaacacctaccttgaaggttctgttagagtggtaacaacttttgattctgagtactgtaggcacggcacttgtgaaagatcagaagctggtgtttgtgtatctactagtggtagatgggtacttaacaatgattattacagatctttaccaggagttttctgtggtgtagatgctgtaaatttacttactaatatgtttacaccactaattcaacctattggtgctttggacatatcagcatctatagtagctggtggtattgtagctatcgtagtaacatgccttgcctactattttatgaggtttagaagagcttttggtgaatacagtcatgtagttgcctttaatactttactattccttatgtcattcactgtactctgtttaacaccagtttactcattcttacctggtgtttattctgttatttacttgtacttgacattttatcttactaatgatgtttcttttttagcacatattcagtggatggttatgttcacacctttagtacctttctggataacaattgcttatatcatttgtatttccacaaagcatttctattggttctttagtaattacctaaagagacgtgtagtctttaatggtgtttcctttagtacttttgaagaagctgcgctgtgcacctttttgttaaataaagaaatgtatctaaagttgcgtagtgatgtgctattacctcttacgcaatataatagatacttagctctttataataagtacaagtattttagtggagcaatggatacaactagctacagagaagctgcttgttgtcatctcgcaaaggctctcaatgacttcagtaactcaggttctgatgttctttaccaaccaccacaaacctctatcacctcagctgttttgcagagtggttttagaaaaatggcattcccatctggtaaagttgagggttgtatggtacaagtaacttgtggtacaactacacttaacggtctttggcttgatgacgtagtttactgtccaagacatgtgatctgcacctctgaagacatgcttaaccctaattatgaagatttactcattcgtaagtctaatcataatttcttggtacaggctggtaatgttcaactcagggttattggacattctatgcaaaattgtgtacttaagcttaaggttgatacagccaatcctaagacacctaagtataagtttgttcgcattcaaccaggacagactttttcagtgttagcttgttacaatggttcaccatctggtgtttaccaatgtgctatgaggcccaatttcactattaagggttcattccttaatggttcatgtggtagtgttggttttaacatagattatgactgtgtctctttttgttacatgcaccatatggaattaccaactggagttcatgctggcacagacttagaaggtaacttttatggaccttttgttgacaggcaaacagcacaagcagctggtacggacacaactattacagttaatgttttagcttggttgtacgctgctgttataaatggagacaggtggtttctcaatcgatttaccacaactcttaatgactttaaccttgtggctatgaagtacaattatgaacctctaacacaagaccatgttgacatactaggacctctttctgctcaaactggaattgccgttttagatatgtgtgcttcattaaaagaattactgcaaaatggtatgaatggacgtaccatattgggtagtgctttattagaagatgaatttacaccttttgatgttgttagacaatgctcaggtgttactttccaaagtgcagtgaaaagaacaatcaagggtacacaccactggttgttactcacaattttgacttcacttttagttttagtccagagtactcaatggtctttgttcttttttttgtatgaaaatgcctttttaccttttgctatgggtattattgctatgtctgcttttgcaatgatgtttgtcaaacataagcatgcatttctctgtttgtttttgttaccttctcttgccactgtagcttattttaatatggtctatatgcctgctagttgggtgatgcgtattatgacatggttggatatggttgatactagtttgtctggttttaagctaaaagactgtgttatgtatgcatcagctgtagtgttactaatccttatgacagcaagaactgtgtatgatgatggtgctaggagagtgtggacacttatgaatgtcttgacactcgtttataaagtttattatggtaatgctttagatcaagccatttccatgtgggctcttataatctctgttacttctaactactcaggtgtagttacaactgtcatgtttttggccagaggtattgtttttatgtgtgttgagtattgccctattttcttcataactggtaatacacttcagtgtataatgctagtttattgtttcttaggctatttttgtacttgttactttggcctcttttgtttactcaaccgctactttagactgactcttggtgtttatgattacttagtttctacacaggagtttagatatatgaattcacagggactactcccacccaagaatagcatagatgccttcaaactcaacattaaattgttgggtgttggtggcaaaccttgtatcaaagtagccactgtacagtctaaaatgtcagatgtaaagtgcacatcagtagtcttactctcagttttgcaacaactcagagtagaatcatcatctaaattgtgggctcaatgtgtccagttacacaatgacattctcttagctaaagatactactgaagcctttgaaaaaatggtttcactactttctgttttgctttccatgcagggtgctgtagacataaacaagctttgtgaagaaatgctggacaacagggcaaccttacaagctatagcctcagagtttagttcccttccatcatatgcagcttttgctactgctcaagaagcttatgagcaggctgttgctaatggtgattctgaagttgttcttaaaaagttgaagaagtctttgaatgtggctaaatctgaatttgaccgtgatgcagccatgcaacgtaagttggaaaagatggctgatcaagctatgacccaaatgtataaacaggctagatctgaggacaagagggcaaaagttactagtgctatgcagacaatgcttttcactatgcttagaaagttggataatgatgcactcaacaacattatcaacaatgcaagagatggttgtgttcccttgaacataatacctcttacaacagcagccaaactaatggttgtcataccagactataacacatataaaaatacgtgtgatggtacaacatttacttatgcatcagcattgtgggaaatccaacaggttgtagatgcagatagtaaaattgttcaacttagtgaaattagtatggacaattcacctaatttagcatggcctcttattgtaacagctttaagggccaattctgctgtcaaattacagaataatgagcttagtcctgttgcactacgacagatgtcttgtgctgccggtactacacaaactgcttgcactgatgacaatgcgttagcttactacaacacaacaaagggaggtaggtttgtacttgcactgttatccgatttacaggatttgaaatgggctagattccctaagagtgatggaactggtactatctatacagaactggaaccaccttgtaggtttgttacagacacacctaaaggtcctaaagtgaagtatttatactttattaaaggattaaacaacctaaatagaggtatggtacttggtagtttagctgccacagtacgtctacaagctggtaatgcaacagaagtgcctgccaattcaactgtattatctttctgtgcttttgctgtagatgctgctaaagcttacaaagattatctagctagtgggggacaaccaatcactaattgtgttaagatgttgtgtacacacactggtactggtcaggcaataacagttacaccggaagccaatatggatcaagaatcctttggtggtgcatcgtgttgtctgtactgccgttgccacatagatcatccaaatcctaaaggattttgtgacttaaaaggtaagtatgtacaaatacctacaacttgtgctaatgaccctgtgggttttacacttaaaaacacagtctgtaccgtctgcggtatgtggaaaggttatggctgtagttgtgatcaactccgcgaacccatgcttcagtcagctgatgcacaatcgtttttaaacgggtttgcggtgtaagtgcagcccgtcttacaccgtgcggcacaggcactagtactgatgtcgtatacagggcttttgacatctacaatgataaagtagctggttttgctaaattcctaaaaactaattgttgtcgcttccaagaaaaggacgaagatgacaatttaattgattcttactttgtagttaagagacacactttctctaactaccaacatgaagaaacaatttataatttacttaaggattgtccagctgttgctaaacatgacttctttaagtttagaatagacggtgacatggtaccacatatatcacgtcaacgtcttactaaatacacaatggcagacctcgtctatgctttaaggcattttgatgaaggtaattgtgacacattaaaagaaatacttgtcacatacaattgttgtgatgatgattatttcaataaaaaggactggtatgattttgtagaaaacccagatatattacgcgtatacgccaacttaggtgaacgtgtacgccaagctttgttaaaaacagtacaattctgtgatgccatgcgaaatgctggtattgttggtgtactgacattagataatcaagatctcaatggtaactggtatgatttcggtgatttcatacaaaccacgccaggtagtggagttcctgttgtagattcttattattcattgttaatgcctatattaaccttgaccagggctttaactgcagagtcacatgttgacactgacttaacaaagccttacattaagtgggatttgttaaaatatgacttcacggaagagaggttaaaactctttgaccgttattttaaatattgggatcagacataccacccaaattgtgttaactgtttggatgacagatgcattctgcattgtgcaaactttaatgttttattctctacagtgttcccacctacaagttttggaccactagtgagaaaaatatttgttgatggtgttccatttgtagtttcaactggataccacttcagagagctaggtgttgtacataatcaggatgtaaacttacatagctctagacttagttttaaggaattacttgtgtatgctgctgaccctgctatgcacgctgcttctggtaatctattactagataaacgcactacgtgcttttcagtagctgcacttactaacaatgttgcttttcaaactgtcaaacccggtaattttaacaaagacttctatgactttgctgtgtctaagggtttctttaaggaaggaagttctgttgaattaaaacacttcttctttgctcaggatggtaatgctgctatcagcgattatgactactatcgttataatctaccaacaatgtgtgatatcagacaactactatttgtagttgaagttgttgataagtactttgattgttacgatggtggctgtattaatgctaaccaagtcatcgtcaacaacctagacaaatcagctggttttccatttaataaatggggtaaggctagactttattatgattcaatgagttatgaggatcaagatgcacttttcgcatatacaaaacgtaatgtcatccctactataactcaaatgaatcttaagtatgccattagtgcaaagaatagagctcgcaccgtagctggtgtctctatctgtagtactatgaccaatagacagtttcatcaaaaattattgaaatcaatagccgccactagaggagctactgtagtaattggaacaagcaaattctatggtggttggcacaacatgttaaaaactgtttatagtgatgtagaaaaccctcaccttatgggttgggattatcctaaatgtgatagagccatgcctaacatgcttagaattatggcctcacttgttcttgctcgcaaacatacaacgtgttgtagcttgtcacaccgtttctatagattagctaatgagtgtgctcaagtattgagtgaaatggtcatgtgtggcggttcactatatgttaaaccaggtggaacctcatcaggagatgccacaactgcttatgctaatagtgtttttaacatttgtcaagctgtcacggccaatgttaatgcacttttatctactgatggtaacaaaattgccgataagtatgtccgcaatttacaacacagactttatgagtgtctctatagaaatagagatgttgacacagactttgtgaatgagttttacgcatatttgcgtaaacatttctcaatgatgatactctctgacgatgctgttgtgtgtttcaatagcacttatgcatctcaaggtctagtggctagcataaagaactttaagtcagttctttattatcaaaacaatgtttttatgtctgaagcaaaatgttggactgagactgaccttactaaaggacctcatgaattttgctctcaacatacaatgctagttaaacagggtgatgattatgtgtaccttccttacccagatccatcaagaatcctaggggccggctgttttgtagatgatatcgtaaaaacagatggtacacttatgattgaacggttcgtgtctttagctatagatgcttacccacttactaaacatcctaatcaggagtatgctgatgtctttcatttgtacttacaatacataagaaagctacatgatgagttaacaggacacatgttagacatgtattctgttatgcttactaatgataacacttcaaggtattgggaacctgagttttatgaggctatgtacacaccgcatacagtcttacaggctgttggggcttgtgttctttgcaattcacagacttcattaagatgtggtgcttgcatacgtagaccattcttatgttgtaaatgctgttacgaccatgtcatatcaacatcacataaattagtcttgtctgttaatccgtatgtttgcaatgctccaggttgtgatgtcacagatgtgactcaactttacttaggaggtatgagctattattgtaaatcacataaaccacccattagttttccattgtgtgctaatggacaagtttttggtttatataaaaatacatgtgttggtagcgataatgttactgactttaatgcaattgcaacatgtgactggacaaatgctggtgattacattttagctaacacctgtactgaaagactcaagctttttgcagcagaaacgctcaaagctactgaggagacatttaaactgtcttatggtattgctactgtacgtgaagtgctgtctgacagagaattacatctttcatgggaagttggtaaacctagaccaccacttaaccgaaattatgtctttactggttatcgtgtaactaaaaacagtaaagtacaaataggagagtacacctttgaaaaaggtgactatggtgatgctgttgtttaccgaggtacaacaacttacaaattaaatgttggtgattattttgtgctgacatcacatacagtaatgccattaagtgcacctacactagtgccacaagagcactatgttagaattactggcttatacccaacactcaatatctcagatgagttttctagcaatgttgcaaattatcaaaaggttggtatgcaaaagtattctacactccagggaccacctggtactggtaagagtcattttgctattggcctagctctctactacccttctgctcgcatagtgtatacagcttgctctcatgccgctgttgatgcactatgtgagaaggcattaaaatatttgcctatagataaatgtagtagaattatacctgcacgtgctcgtgtagagtgttttgataaattcaaagtgaattcaacattagaacagtatgtcttttgtactgtaaatgcattgcctgagacgacagcagatatagttgtctttgatgaaatttcaatggccacaaattatgatttgagtgttgtcaatgccagattacgtgctaagcactatgtgtacattggcgaccctgctcaattacctgcaccacgcacattgctaactaagggcacactagaaccagaatatttcaattcagtgtgtagacttatgaaaactataggtccagacatgttcctcggaacttgtcggcgttgtcctgctgaaattgttgacactgtgagtgctttggtttatgataataagcttaaagcacataaagacaaatcagctcaatgctttaaaatgttttataagggtgttatcacgcatgatgtttcatctgcaattaacaggccacaaataggcgtggtaagagaattccttacacgtaaccctgcttggagaaaagctgtctttatttcaccttataattcacagaatgctgtagcctcaaagattttgggactaccaactcaaactgttgattcatcacagggctcagaatatgactatgtcatattcactcaaaccactgaaacagctcactcttgtaatgtaaacagatttaatgttgctattaccagagcaaaagtaggcatactttgcataatgtctgatagagacctttatgacaagttgcaatttacaagtcttgaaattccacgtaggaatgtggcaactttacaagctgaaaatgtaacaggactctttaaagattgtagtaaggtaatcactgggttacatcctacacaggcacctacacacctcagtgttgacactaaattcaaaactgaaggtttatgtgttgacatacctggcatacctaaggacatgacctatagaagactcatctctatgatgggttttaaaatgaattatcaagttaatggttaccctaacatgtttatcacccgcgaagaagctataagacatgtacgtgcatggattggcttcgatgtcgaggggtgtcatgctactagagaagctgttggtaccaatttacctttacagctaggtttttctacaggtgttaacctagttgctgtacctacaggttatgttgatacacctaataatacagatttttccagagttagtgctaaaccaccgcctggagatcaatttaaacacctcataccacttatgtacaaaggacttccttggaatgtagtgcgtataaagattgtacaaatgttaagtgacacacttaaaaatctctctgacagagtcgtatttgtcttatgggcacatggctttgagttgacatctatgaagtattttgtgaaaataggacctgagcgcacctgttgtctatgtgatagacgtgccacatgcttttccactgcttcagacacttatgcctgttggcatcattctattggatttgattacgtctataatccgtttatgattgatgttcaacaatggggttttacaggtaacctacaaagcaaccatgatctgtattgtcaagtccatggtaatgcacatgtagctagttgtgatgcaatcatgactaggtgtctagctgtccacgagtgctttgttaagcgtgttgactggactattgaatatcctataattggtgatgaactgaagattaatgcggcttgtagaaaggttcaacacatggttgttaaagctgcattattagcagacaaattcccagttcttcacgacattggtaaccctaaagctattaagtgtgtacctcaagctgatgtagaatggaagttctatgatgcacagccttgtagtgacaaagcttataaaatagaagaattattctattcttatgccacacattctgacaaattcacagatggtgtatgcctattttggaattgcaatgtcgatagatatcctgctaattccattgtttgtagatttgacactagagtgctatctaaccttaacttgcctggttgtgatggtggcagtttgtatgtaaataaacatgcattccacacaccagcttttgataaaagtgcttttgttaatttaaaacaattaccatttttctattactctgacagtccatgtgagtctcatggaaaacaagtagtgtcagatatagattatgtaccactaaagtctgctacgtgtataacacgttgcaatttaggtggtgctgtctgtagacatcatgctaatgagtacagattgtatctcgatgcttataacatgatgatctcagctggctttagcttgtgggtttacaaacaatttgatacttataacctctggaacacttttacaagacttcagagtttagaaaatgtggcttttaatgttgtaaataagggacactttgatggacaacagggtgaagtaccagtttctatcattaataacactgtttacacaaaagttgatggtgttgatgtagaattgtttgaaaataaaacaacattacctgttaatgtagcatttgagctttgggctaagcgcaacattaaaccagtaccagaggtgaaaatactcaataatttgggtgtggacattgctgctaatactgtgatctgggactacaaaagagatgctccagcacatatatctactattggtgtttgttctatgactgacatagccaagaaaccaactgaaacgatttgtgcaccactcactgtcttttttgatggtagagttgatggtcaagtagacttatttagaaatgcccgtaatggtgttcttattacagaaggtagtgttaaaggtttacaaccatctgtaggtcccaaacaagctagtcttaatggagtcacattaattggagaagccgtaaaaacacagttcaattattataagaaagttgatggtgttgtccaacaattacctgaaacttactttactcagagtagaaatttacaagaatttaaacccaggagtcaaatggaaattgatttcttagaattagctatggatgaattcattgaacggtataaattagaaggctatgccttcgaacatatcgtttatggagattttagtcatagtcagttaggtggtttacatctactgattggactagctaaacgttttaaggaatcaccttttgaattagaagattttattcctatggacagtacagttaaaaactatttcataacagatgcgcaaacaggttcatctaagtgtgtgtgttctgttattgatttattacttgatgattttgttgaaataataaaatcccaagatttatctgtagtttctaaggttgtcaaagtgactattgactatacagaaatttcatttatgctttggtgtaaagatggccatgtagaaacattttacccaaaattacaatctagtcaagcgtggcaaccgggtgttgctatgcctaatctttacaaaatgcaaagaatgctattagaaaagtgtgaccttcaaaattatggtgatagtgcaacattacctaaaggcataatgatgaatgtcgcaaaatatactcaactgtgtcaatatttaaacacattaacattagctgtaccctataatatgagagttatacattttggtgctggttctgataaaggagttgcaccaggtacagctgttttaagacagtggttgcctacgggtacgctgcttgtcgattcagatcttaatgactttgtctctgatgcagattcaactttgattggtgattgtgcaactgtacatacagctaataaatgggatctcattattagtgatatgtacgaccctaagactaaaaatgttacaaaagaaaatgactctaaagagggttttttcacttacatttgtgggtttatacaacaaaagctagctcttggaggttccgtggctataaagataacagaacattcttggaatgctgatctttataagctcatgggacacttcgcatggtggacagcctttgttactaatgtgaatgcgtcatcatctgaagcatttttaattggatgtaattatcttggcaaaccacgcgaacaaatagatggttatgtcatgcatgcaaattacatattttggaggaatacaaatccaattcagttgtcttcctattctttatttgacatgagtaaatttccccttaaattaaggggtactgctgttatgtctttaaaagaaggtcaaatcaatgatatgattttatctcttcttagtaaaggtagacttataattagagaaaacaacagagttgttatttctagtgatgttcttgttaacaactaaacgaacaatgtttgtttttcttgttttattgccactagtctctagtcagtgtgttaatcttacaaccagaactcaattaccccctgcatacactaattctttcacacgtggtgtttattaccctgacaaagttttcagatcctcagttttacattcaactcaggacttgttcttacctttcttttccaatgttacttggttccatgctatacatgtctctgggaccaatggtactaagaggtttgataaccctgtcctaccatttaatgatggtgtttattttgcttccactgagaagtctaacataataagaggctggatttttggtactactttagattcgaagacccagtccctacttattgttaataacgctactaatgttgttattaaagtctgtgaatttcaattttgtaatgatccatttttgggtgtttattaccacaaaaacaacaaaagttggatggaaagtgagttcagagtttattctagtgcgaataattgcacttttgaatatgtctctcagccttttcttatggaccttgaaggaaaacagggtaatttcaaaaatcttagggaatttgtgtttaagaatattgatggttattttaaaatatattctaagcacacgcctattaatttagtgcgtgatctccctcagggtttttcggctttagaaccattggtagatttgccaataggtattaacatcactaggtttcaaactttacttgctttacatagaagttatttgactcctggtgattcttcttcaggttggacagctggtgctgcagcttattatgtgggttatcttcaacctaggacttttctattaaaatataatgaaaatggaaccattacagatgctgtagactgtgcacttgaccctctctcagaaacaaagtgtacgttgaaatccttcactgtagaaaaaggaatctatcaaacttctaactttagagtccaaccaacagaatctattgttagatttcctaatattacaaacttgtgcccttttggtgaagtttttaacgccaccagatttgcatctgtttatgcttggaacaggaagagaatcagcaactgtgttgctgattattctgtcctatataattccgcatcattttccacttttaagtgttatggagtgtctcctactaaattaaatgatctctgctttactaatgtctatgcagattcatttgtaattagaggtgatgaagtcagacaaatcgctccagggcaaactggaaagattgctgattataattataaattaccagatgattttacaggctgcgttatagcttggaattctaacaatcttgattctaaggttggtggtaattataattacctgtatagattgtttaggaagtctaatctcaaaccttttgagagagatatttcaactgaaatctatcaggccggtagcacaccttgtaatggtgttgaaggttttaattgttactttcctttacaatcatatggtttccaacccactaatggtgttggttaccaaccatacagagtagtagtactttcttttgaacttctacatgcaccagcaactgtttgtggacctaaaaagtctactaatttggttaaaaacaaatgtgtcaatttcaacttcaatggtttaacaggcacaggtgttcttactgagtctaacaaaaagtttctgcctttccaacaatttggcagagacattgctgacactactgatgctgtccgtgatccacagacacttgagattcttgacattacaccatgttcttttggtggtgtcagtgttataacaccaggaacaaatacttctaaccaggttgctgttctttatcaggatgttaactgcacagaagtccctgttgctattcatgcagatcaacttactcctacttggcgtgtttattctacaggttctaatgtttttcaaacacgtgcaggctgtttaataggggctgaacatgtcaacaactcatatgagtgtgacatacccattggtgcaggtatatgcgctagttatcagactcagactaattctcctcggcgggcacgtagtgtagctagtcaatccatcattgcctacactatgtcacttggtgcagaaaattcagttgcttactctaataactctattgccatacccacaaattttactattagtgttaccacagaaattctaccagtgtctatgaccaagacatcagtagattgtacaatgtacatttgtggtgattcaactgaatgcagcaatcttttgttgcaatatggcagtttttgtacacaattaaaccgtgctttaactggaatagctgttgaacaagacaaaaacacccaagaagtttttgcacaagtcaaacaaatttacaaaacaccaccaattaaagattttggtggttttaatttttcacaaatattaccagatccatcaaaaccaagcaagaggtcatttattgaagatctacttttcaacaaagtgacacttgcagatgctggcttcatcaaacaatatggtgattgccttggtgatattgctgctagagacctcatttgtgcacaaaagtttaacggccttactgttttgccacctttgctcacagatgaaatgattgctcaatacacttctgcactgttagcgggtacaatcacttctggttggacctttggtgcaggtgctgcattacaaataccatttgctatgcaaatggcttataggtttaatggtattggagttacacagaatgttctctatgagaaccaaaaattgattgccaaccaatttaatagtgctattggcaaaattcaagactcactttcttccacagcaagtgcacttggaaaacttcaagatgtggtcaaccaaaatgcacaagctttaaacacgcttgttaaacaacttagctccaattttggtgcaatttcaagtgttttaaatgatatcctttcacgtcttgacaaagttgaggctgaagtgcaaattgataggttgatcacaggcagacttcaaagtttgcagacatatgtgactcaacaattaattagagctgcagaaatcagagcttctgctaatcttgctgctactaaaatgtcagagtgtgtacttggacaatcaaaaagagttgatttttgtggaaagggctatcatcttatgtccttccctcagtcagcacctcatggtgtagtcttcttgcatgtgacttatgtccctgcacaagaaaagaacttcacaactgctcctgccatttgtcatgatggaaaagcacactttcctcgtgaaggtgtctttgtttcaaatggcacacactggtttgtaacacaaaggaatttttatgaaccacaaatcattactacagacaacacatttgtgtctggtaactgtgatgttgtaataggaattgtcaacaacacagtttatgatcctttgcaacctgaattagactcattcaaggaggagttagataaatattttaagaatcatacatcaccagatgttgatttaggtgacatctctggcattaatgcttcagttgtaaacattcaaaaagaaattgaccgcctcaatgaggttgccaagaatttaaatgaatctctcatcgatctccaagaacttggaaagtatgagcagtatataaaatggccatggtacatttggctaggttttatagctggcttgattgccatagtaatggtgacaattatgctttgctgtatgaccagttgctgtagttgtctcaagggctgttgttcttgtggatcctgctgcaaatttgatgaagacgactctgagccagtgctcaaaggagtcaaattacattacacataaacgaacttatggatttgtttatgagaatcttcacaattggaactgtaactttgaagcaaggtgaaatcaaggatgctactccttcagattttgttcgcgctactgcaacgataccgatacaagcctcactccctttcggatggcttattgttggcgttgcacttcttgctgtttttcagagcgcttccaaaatcataaccctcaaaaagagatggcaactagcactctccaagggtgttcactttgtttgcaacttgctgttgttgtttgtaacagtttactcacaccttttgctcgttgctgctggccttgaagccccttttctctatctttatgctttagtctacttcttgcagagtataaactttgtaagaataataatgaggctttggctttgctggaaatgccgttccaaaaacccattactttatgatgccaactattttctttgctggcatactaattgttacgactattgtataccttacaatagtgtaacttcttcaattgtcattacttcaggtgatggcacaacaagtcctatttctgaacatgactaccagattggtggttatactgaaaaatgggaatctggagtaaaagactgtgttgtattacacagttacttcacttcagactattaccagctgtactcaactcaattgagtacagacactggtgttgaacatgttaccttcttcatctacaataaaattgttgatgagcctgaagaacatgtccaaattcacacaatcgacggttcatccggagttgttaatccagtaatggaaccaatttatgatgaaccgacgacgactactagcgtgcctttgtaagcacaagctgatgagtacgaacttatgtactcattcgtttcggaagagacaggtacgttaatagttaatagcgtacttctttttcttgctttcgtggtattcttgctagttacactagccatccttactgcgcttcgattgtgtgcgtactgctgcaatattgttaacgtgagtcttgtaaaaccttctttttacgtttactctcgtgttaaaaatctgaattcttctagagttcctgatcttctggtctaaacgaactaaatattatattagtttttctgtttggaactttaattttagccatggcagattccaacggtactattaccgttgaagagcttaaaaagctccttgaacaatggaacctagtaataggtttcctattccttacatggatttgtcttctacaatttgcctatgccaacaggaataggtttttgtatataattaagttaattttcctctggctgttatggccagtaactttagcttgttttgtgcttgctgctgtttacagaataaattggatcaccggtggaattgctatcgcaatggcttgtcttgtaggcttgatgtggctcagctacttcattgcttctttcagactgtttgcgcgtacgcgttccatgtggtcattcaatccagaaactaacattcttctcaacgtgccactccatggcactattctgaccagaccgcttctagaaagtgaactcgtaatcggagctgtgatccttcgtggacatcttcgtattgctggacaccatctaggacgctgtgacatcaaggacctgcctaaagaaatcactgttgctacatcacgaacgctttcttattacaaattgggagcttcgcagcgtgtagcaggtgactcaggttttgctgcatacagtcgctacaggattggcaactataaattaaacacagaccattccagtagcagtgacaatattgctttgcttgtacagtaagtgacaacagatgtttcatctcgttgactttcaggttactatagcagagatattactaattattatgaggacttttaaagtttccatttggaatcttgattacatcataaacctcataattaaaaatttatctaagtcactaactgagaataaatattctcaattagatgaagagcaaccaatggagattgattaaacgaacatgaaaattattcttttcttggcactgataacactcgctacttgtgagctttatcactaccaagagtgtgttagaggtacaacagtacttttaaaagaaccttgctcttctggaacatacgagggcaattcaccatttcatcctctagctgataacaaatttgcactgacttgctttagcactcaatttgcttttgcttgtcctgacggcgtaaaacacgtctatcagttacgtgccagatcagtttcacctaaactgttcatcagacaagaggaagttcaagaactttactctccaatttttcttattgttgcggcaatagtgtttataacactttgcttcacactcaaaagaaagacagaatgattgaactttcattaattgacttctatttgtgctttttagcctttctgctattccttgttttaattatgcttattatcttttggttctcacttgaactgcaagatcataatgaaacttgtcacgcctaaacgaacatgaaatttcttgttttcttaggaatcatcacaactgtagctgcatttcaccaagaatgtagtttacagtcatgtactcaacatcaaccatatgtagttgatgacccgtgtcctattcacttctattctaaatggtatattagagtaggagctagaaaatcagcacctttaattgaattgtgcgtggatgaggctggttctaaatcacccattcagtacatcgatatcggtaattatacagtttcctgtttaccttttacaattaattgccaggaacctaaattgggtagtcttgtagtgcgttgttcgttctatgaagactttttagagtatcatgacgttcgtgttgttttagatttcatctaaacgaacaaactaaaatgtctgataatggaccccaaaatcagcgaaatgcaccccgcattacgtttggtggaccctcagattcaactggcagtaaccagaatggagaacgcagtggggcgcgatcaaaacaacgtcggccccaaggtttacccaataatactgcgtcttggttcaccgctctcactcaacatggcaaggaagaccttaaattccctcgaggacaaggcgttccaattaacaccaatagcagtccagatgaccaaattggctactaccgaagagctaccagacgaattcgtggtggtgacggtaaaatgaaagatctcagtccaagatggtatttctactacctaggaactgggccagaagctggacttccctatggtgctaacaaagacggcatcatatgggttgcaactgagggagccttgaatacaccaaaagatcacattggcacccgcaatcctgctaacaatgctgcaatcgtgctacaacttcctcaaggaacaacattgccaaaaggcttctacgcagaagggagcagaggcggcagtcaagcctcttctcgttcctcatcacgtagtcgcaacagttcaagaaattcaactccaggcagcagtaggggaacttctcctgctagaatggctggcaatggcggtgatgctgctcttgctttgctgctgcttgacagattgaaccagcttgagagcaaaatgtctggtaaaggccaacaacaacaaggccaaactgtcactaagaaatctgctgctgaggcttctaagaagcctcggcaaaaacgtactgccactaaagcatacaatgtaacacaagctttcggcagacgtggtccagaacaaacccaaggaaattttggggaccaggaactaatcagacaaggaactgattacaaacattggccgcaaattgcacaatttgcccccagcgcttcagcgttcttcggaatgtcgcgcattggcatggaagtcacaccttcgggaacgtggttgacctacacaggtgccatcaaattggatgacaaagatccaaatttcaaagatcaagtcattttgctgaataagcatattgacgcatacaaaacattcccaccaacagagcctaaaaaggacaaaaagaagaaggctgatgaaactcaagccttaccgcagagacagaagaaacagcaaactgtgactcttcttcctgctgcagatttggatgatttctccaaacaattgcaacaatccatgagcagtgctgactcaactcaggcctaaactcatgcagaccacacaaggcagatgggctatataaacgttttcgcttttccgtttacgatatatagtctactcttgtgcagaatgaattctcgtaactacatagcacaagtagatgtagttaactttaatctcacatagcaatctttaatcagtgtgtaacattagggaggacttgaaagagccaccacattttcaccgaggccacgcggagtacgatcgagtgtacagtgaacaatgctagggagagctgcctatatggaagagccctaatgtgtaaaattaattttagtagtgctatccccatgtgattttaatagcttcttaggagaatgacaaaaaaaaaaaaaaaaaaaaaaaaaaaaaaaaa

SEQ ID NO: 2 - protein, 1273 aa, SARS-CoV-2
  REGION 1..1273: note = SARS-CoV-2 spike protein with native signal peptide
MFVFLVLLPLVSSQCVNLTTRTQLPPAYTNSFTRGVYYPDKVFRSSVLHSTQDLFLPFFSNVTWFHAIHVSGTNGTKRFDNPVLPFNDGVYFASTEKSNIIRGWIFGTTLDSKTQSLLIVNNATNVVIKVCEFQFCNDPFLGVYYHKNNKSWMESEFRVYSSANNCTFEYVSQPFLMDLEGKQGNFKNLREFVFKNIDGYFKIYSKHTPINLVRDLPQGFSALEPLVDLPIGINITRFQTLLALHRSYLTPGDSSSGWTAGAAAYYVGYLQPRTFLLKYNENGTITDAVDCALDPLSETKCTLKSFTVEKGIYQTSNFRVQPTESIVRFPNITNLCPFGEVFNATRFASVYAWNRKRISNCVADYSVLYNSASFSTFKCYGVSPTKLNDLCFTNVYADSFVIRGDEVRQIAPGQTGKIADYNYKLPDDFTGCVIAWNSNNLDSKVGGNYNYLYRLFRKSNLKPFERDISTEIYQAGSTPCNGVEGFNCYFPLQSYGFQPTNGVGYQPYRVVVLSFELLHAPATVCGPKKSTNLVKNKCVNFNFNGLTGTGVLTESNKKFLPFQQFGRDIADTTDAVRDPQTLEILDITPCSFGGVSVITPGTNTSNQVAVLYQDVNCTEVPVAIHADQLTPTWRVYSTGSNVFQTRAGCLIGAEHVNNSYECDIPIGAGICASYQTQTNSPRRARSVASQSIIAYTMSLGAENSVAYSNNSIAIPTNFTISVTTEILPVSMTKTSVDCTMYICGDSTECSNLLLQYGSFCTQLNRALTGIAVEQDKNTQEVFAQVKQIYKTPPIKDFGGFNFSQILPDPSKPSKRSFIEDLLFNKVTLADAGFIKQYGDCLGDIAARDLICAQKFNGLTVLPPLLTDEMIAQYTSALLAGTITSGWTFGAGAALQIPFAMQMAYRFNGIGVTQNVLYENQKLIANQFNSAIGKIQDSLSSTASALGKLQDVVNQNAQALNTLVKQLSSNFGAISSVLNDILSRLDKVEAEVQIDRLITGRLQSLQTYVTQQLIRAAEIRASANLAATKMSECVLGQSKRVDFCGKGYHLMSFPQSAPHGVVFLHVTYVPAQEKNFTTAPAICHDGKAHFPREGVFVSNGTHWFVTQRNFYEPQIITTDNTFVSGNCDVVIGIVNNTVYDPLQPELDSFKEELDKYFKNHTSPDVDLGDISGINASVVNIQKEIDRLNEVAKNLNESLIDLQELGKYEQYIKWPWYIWLGFIAGLIAIVMVTIMLCCMTSCCSCLKGCCSCGSCCKFDEDDSEPVLKGVKLHYT

SEQ ID NO: 3 - DNA, 3819 bp, SARS-CoV-2
  misc_feature 1..3819: note = SARS-CoV-2 spike protein with native signal peptide
  source 1..3819: mol_type = other DNA
atgtttgtttttcttgttttattgccattagtctctagtcagtgtgttaatcttacaaccagaactcaattaccccctgcatacactaattctttcacacgtggtgtttattaccctgacaaagttttcagatcctcagttttacattcaactcaggacttgttcttacctttcttttccaatgttacttggttccatgctatacatgtctctgggaccaatggtactaagaggtttgataaccctgtcctaccatttaatgatggtgtttattttgcttccactgagaagtctaacataataagaggctggatttttggtactactttagattcgaagacccagtccctacttattgttaataacgctactaatgttgttattaaagtctgtgaatttcaattttgtaatgatccatttttgggtgtttattaccacaaaaacaacaaaagttggatggaaagtgagttcagagtttattctagtgcgaataattgcacttttgaatatgtctctcagccttttcttatggaccttgaaggaaaacagggtaatttcaaaaatcttagggaatttgtgtttaagaatattgatggttattttaaaatatattctaagcacacgcctattaatttagtgcgtgatctccctcagggtttttcggctttagaaccattggtagatttgccaataggtattaacatcactaggtttcaaactttacttgctttacatagaagttatttgactcctggtgattcttcttcaggttggacagctggtgctgcagcttattatgtgggttatcttcaacctaggacttttctattaaaatataatgaaaatggaaccattacagatgctgtagactgtgcacttgaccctctctcagaaacaaagtgtacgttgaaatccttcactgtagaaaaaggaatctatcaaacttctaactttagagtccaaccaacagaatctattgttagatttcctaatattacaaacttgtgcccttttggtgaagtttttaacgccaccagatttgcatctgtttatgcttggaacaggaagagaatcagcaactgtgttgctgattattctgtcctatataattccgcatcattttccacttttaagtgttatggagtgtctcctactaaattaaatgatctctgctttactaatgtctatgcagattcatttgtaattagaggtgatgaagtcagacaaatcgctccagggcaaactggaaagattgctgattataattataaattaccagatgattttacaggctgcgttatagcttggaattctaacaatcttgattctaaggttggtggtaattataattacctgtatagattgtttaggaagtctaatctcaaaccttttgagagagatatttcaactgaaatctatcaggccggtagcacaccttgtaatggtgttgaaggttttaattgttactttcctttacaatcatatggtttccaacccactaatggtgttggttaccaaccatacagagtagtagtactttcttttgaacttctacatgcaccagcaactgtttgtggacctaaaaagtctactaatttggttaaaaacaaatgtgtcaatttcaacttcaatggtttaacaggcacaggtgttcttactgagtctaacaaaaagtttctgcctttccaacaatttggcagagacattgctgacactactgatgctgtccgtgatccacagacacttgagattcttgacattacaccatgttcttttggtggtgtcagtgttataacaccaggaacaaatacttctaaccaggttgctgttctttatcaggatgttaactgcacagaagtccctgttgctattcatgcagatcaacttactcctacttggcgtgtttattctacaggttctaatgtttttcaaacacgtgcaggctgtttaataggggctgaacatgtcaacaactcatatgagtgtgacatacccattggtgcaggtatatgcgctagttatcagactcagactaattctcctcggcgggcacgtagtgtagctagtcaatccatcattgcctacactatgtcacttggtgcagaaaattcagttgcttactctaataactctattgccatacccacaaattttactattagtgttaccacagaaattctaccagtgtctatgaccaagacatcagtagattgtacaatgtacatttgtggtgattcaactgaatgcagcaatcttttgttgcaatatggcagtttttgtacacaattaaaccgtgctttaactggaatagctgttgaacaagacaaaaacacccaagaagtttttgcacaagtcaaacaaatttacaaaacaccaccaattaaagattttggtggttttaatttttcacaaatattaccagatccatcaaaaccaagcaagaggtcatttattgaagatctacttttcaacaaagtgacacttgcagatgctggcttcatcaaacaatatggtgattgccttggtgatattgctgctagagacctcatttgtgcacaaaagtttaacggccttactgttttgccacctttgctcacagatgaaatgattgctcaatacacttctgcactgttagcgggtacaatcacttctggttggacctttggtgcaggtgctgcattacaaataccatttgctatgcaaatggcttataggtttaatggtattggagttacacagaatgttctctatgagaaccaaaaattgattgccaaccaatttaatagtgctattggcaaaattcaagactcactttcttccacagcaagtgcacttggaaaacttcaagatgtggtcaaccaaaatgcacaagctttaaacacgcttgttaaacaacttagctccaattttggtgcaatttcaagtgttttaaatgatatcctttcacgtcttgacaaagttgaggctgaagtgcaaattgataggttgatcacaggcagacttcaaagtttgcagacatatgtgactcaacaattaattagagctgcagaaatcagagcttctgctaatcttgctgctactaaaatgtcagagtgtgtacttggacaatcaaaaagagttgatttttgtggaaagggctatcatcttatgtccttccctcagtcagcacctcatggtgtagtcttcttgcatgtgacttatgtccctgcacaagaaaagaacttcacaactgctcctgccatttgtcatgatggaaaagcacactttcctcgtgaaggtgtctttgtttcaaatggcacacactggtttgtaacacaaaggaatttttatgaaccacaaatcattactacagacaacacatttgtgtctggtaactgtgatgttgtaataggaattgtcaacaacacagtttatgatcctttgcaacctgaattagactcattcaaggaggagttagataaatattttaagaatcatacatcaccagatgttgatttaggtgacatctctggcattaatgcttcagttgtaaacattcaaaaagaaattgaccgcctcaatgaggttgccaagaatttaaatgaatctctcatcgatctccaagaacttggaaagtatgagcagtatataaaatggccatggtacatttggctaggttttatagctggcttgattgccatagtaatggtgacaattatgctttgctgtatgaccagttgctgtagttgtctcaagggctgttgttcttgtggatcctgctgcaaatttgatgaagacgactctgagccagtgctcaaaggagtcaaattacattacaca

SEQ ID NO: 4 - protein, 1198 aa, SARS-CoV-2
  REGION 1..1198: note = SARS-CoV-2 spike protein ectodomain (ECD)
QCVNLTTRTQLPPAYTNSFTRGVYYPDKVFRSSVLHSTQDLFLPFFSNVTWFHAIHVSGTNGTKRFDNPVLPFNDGVYFASTEKSNIIRGWIFGTTLDSKTQSLLIVNNATNVVIKVCEFQFCNDPFLGVYYHKNNKSWMESEFRVYSSANNCTFEYVSQPFLMDLEGKQGNFKNLREFVFKNIDGYFKIYSKHTPINLVRDLPQGFSALEPLVDLPIGINITRFQTLLALHRSYLTPGDSSSGWTAGAAAYYVGYLQPRTFLLKYNENGTITDAVDCALDPLSETKCTLKSFTVEKGIYQTSNFRVQPTESIVRFPNITNLCPFGEVFNATRFASVYAWNRKRISNCVADYSVLYNSASFSTFKCYGVSPTKLNDLCFTNVYADSFVIRGDEVRQIAPGQTGKIADYNYKLPDDFTGCVIAWNSNNLDSKVGGNYNYLYRLFRKSNLKPFERDISTEIYQAGSTPCNGVEGFNCYFPLQSYGFQPTNGVGYQPYRVVVLSFELLHAPATVCGPKKSTNLVKNKCVNFNFNGLTGTGVLTESNKKFLPFQQFGRDIADTTDAVRDPQTLEILDITPCSFGGVSVITPGTNTSNQVAVLYQDVNCTEVPVAIHADQLTPTWRVYSTGSNVFQTRAGCLIGAEHVNNSYECDIPIGAGICASYQTQTNSPRRARSVASQSIIAYTMSLGAENSVAYSNNSIAIPTNFTISVTTEILPVSMTKTSVDCTMYICGDSTECSNLLLQYGSFCTQLNRALTGIAVEQDKNTQEVFAQVKQIYKTPPIKDFGGFNFSQILPDPSKPSKRSFIEDLLFNKVTLADAGFIKQYGDCLGDIAARDLICAQKFNGLTVLPPLLTDEMIAQYTSALLAGTITSGWTFGAGAALQIPFAMQMAYRFNGIGVTQNVLYENQKLIANQFNSAIGKIQDSLSSTASALGKLQDVVNQNAQALNTLVKQLSSNFGAISSVLNDILSRLDKVEAEVQIDRLITGRLQSLQTYVTQQLIRAAEIRASANLAATKMSECVLGQSKRVDFCGKGYHLMSFPQSAPHGVVFLHVTYVPAQEKNFTTAPAICHDGKAHFPREGVFVSNGTHWFVTQRNFYEPQIITTDNTFVSGNCDVVIGIVNNTVYDPLQPELDSFKEELDKYFKNHTSPDVDLGDISGINASVVNIQKEIDRLNEVAKNLNESLIDLQELGKYEQYIK

SEQ ID NO: 5 - DNA, 3594 bp, SARS-CoV-2
  misc_feature 1..3594: note = SARS-CoV-2 spike protein ECD coding sequence
  source 1..3594: mol_type = other DNA
cagtgtgttaatcttacaaccagaactcaattaccccctgcatacactaattctttcacacgtggtgtttattaccctgacaaagttttcagatcctcagttttacattcaactcaggacttgttcttacctttcttttccaatgttacttggttccatgctatacatgtctctgggaccaatggtactaagaggtttgataaccctgtcctaccatttaatgatggtgtttattttgcttccactgagaagtctaacataataagaggctggatttttggtactactttagattcgaagacccagtccctacttattgttaataacgctactaatgttgttattaaagtctgtgaatttcaattttgtaatgatccatttttgggtgtttattaccacaaaaacaacaaaagttggatggaaagtgagttcagagtttattctagtgcgaataattgcacttttgaatatgtctctcagccttttcttatggaccttgaaggaaaacagggtaatttcaaaaatcttagggaatttgtgtttaagaatattgatggttattttaaaatatattctaagcacacgcctattaatttagtgcgtgatctccctcagggtttttcggctttagaaccattggtagatttgccaataggtattaacatcactaggtttcaaactttacttgctttacatagaagttatttgactcctggtgattcttcttcaggttggacagctggtgctgcagcttattatgtgggttatcttcaacctaggacttttctattaaaatataatgaaaatggaaccattacagatgctgtagactgtgcacttgaccctctctcagaaacaaagtgtacgttgaaatccttcactgtagaaaaaggaatctatcaaacttctaactttagagtccaaccaacagaatctattgttagatttcctaatattacaaacttgtgcccttttggtgaagtttttaacgccaccagatttgcatctgtttatgcttggaacaggaagagaatcagcaactgtgttgctgattattctgtcctatataattccgcatcattttccacttttaagtgttatggagtgtctcctactaaattaaatgatctctgctttactaatgtctatgcagattcatttgtaattagaggtgatgaagtcagacaaatcgctccagggcaaactggaaagattgctgattataattataaattaccagatgattttacaggctgcgttatagcttggaactctaacaatcttgattctaaggttggtggtaattataattacctgtatagattgtttaggaagtctaatctcaaaccttttgagagagatatttcaactgaaatctatcaggccggtagcacaccttgtaatggtgttgaaggttttaattgttactttcctttacaatcatatggtttccaacccactaatggtgttggttaccaaccatacagagtagtagtactttcttttgaacttctacatgcaccagcaactgtttgtggacctaaaaagtctactaatttggttaaaaacaaatgtgtcaatttcaacttcaatggtttaacaggcacaggtgttcttactgagtctaacaaaaagtttctgcctttccaacaatttggcagagacattgctgacactactgatgctgtccgtgatccacagacacttgagattcttgacattacaccatgttcttttggtggtgtcagtgttataacaccaggaacaaatacttctaaccaggttgctgttctttatcaggatgttaactgcacagaagtccctgttgctattcatgcagatcaacttactcctacttggcgtgtttattctacaggttctaatgtttttcaaacacgtgcaggctgtttaataggggctgaacatgtcaacaactcatatgagtgtgacatacccattggtgcaggtatatgcgctagttatcagactcagactaattctcctcggcgggcacgtagtgtagctagtcaatccatcattgcctacactatgtcacttggtgcagaaaattcagttgcttactctaataactctattgccatacccacaaattttactattagtgttaccacagaaattctaccagtgtctatgaccaagacatcagtagattgtacaatgtacatttgtggtgattcaactgaatgcagcaatcttttgttgcaatatggcagtttttgtacacaattaaaccgtgctttaactggaatagctgttgaacaagacaaaaacacccaagaagtttttgcacaagtcaaacaaatttacaaaacaccaccaattaaagattttggtggttttaatttttcacaaatattaccagatccatcaaaaccaagcaagaggtcatttattgaagatctacttttcaacaaagtgacacttgcagatgctggcttcatcaaacaatatggtgattgccttggtgatattgctgctagagacctcatttgtgcacaaaagtttaacggccttactgttttgccacctttgctcacagatgaaatgattgctcaatacacttctgcactgttagcgggtacaatcacttctggttggacctttggtgcaggtgctgcattacaaataccatttgctatgcaaatggcttataggtttaatggtattggagttacacagaatgttctctatgagaaccaaaaattgattgccaaccaatttaatagtgctattggcaaaattcaagactcactttcttccacagcaagtgcacttggaaaacttcaagatgtggtcaaccaaaatgcacaagctttaaacacgcttgttaaacaacttagctccaattttggtgcaatttcaagtgttttaaatgatatcctttcacgtcttgacaaagttgaggctgaagtgcaaattgataggttgatcacaggcagacttcaaagtttgcagacatatgtgactcaacaattaattagagctgcagaaatcagagcttctgctaatcttgctgctactaaaatgtcagagtgtgtacttggacaatcaaaaagagttgatttttgtggaaagggctatcatcttatgtccttccctcagtcagcacctcatggtgtagtcttcttgcatgtgacttatgtccctgcacaagaaaagaacttcacaactgctcctgccatttgtcatgatggaaaagcacactttcctcgtgaaggtgtctttgtttcaaatggcacacactggtttgtaacacaaaggaatttttatgaaccacaaatcattactacagacaacacatttgtgtctggtaactgtgatgttgtaataggaattgtcaacaacacagtttatgatcctttgcaacctgaattagactcattcaaggaggagttagataaatattttaagaatcatacatcaccagatgttgatttaggtgacatctctggcattaatgcttcagttgtaaacattcaaaaagaaattgaccgcctcaatgaggttgccaagaatttaaatgaatctctcatcgatctccaagaacttggaaagtatgagcagtatataaaa

SEQ ID NO: 6 - protein, 672 aa, SARS-CoV-2
  REGION 1..672: note = SARS-CoV-2 spike protein S1 subunit
QCVNLTTRTQLPPAYTNSFTRGVYYPDKVFRSSVLHSTQDLFLPFFSNVTWFHAIHVSGTNGTKRFDNPVLPFNDGVYFASTEKSNIIRGWIFGTTLDSKTQSLLIVNNATNVVIKVCEFQFCNDPFLGVYYHKNNKSWMESEFRVYSSANNCTFEYVSQPFLMDLEGKQGNFKNLREFVFKNIDGYFKIYSKHTPINLVRDLPQGFSALEPLVDLPIGINITRFQTLLALHRSYLTPGDSSSGWTAGAAAYYVGYLQPRTFLLKYNENGTITDAVDCALDPLSETKCTLKSFTVEKGIYQTSNFRVQPTESIVRFPNITNLCPFGEVFNATRFASVYAWNRKRISNCVADYSVLYNSASFSTFKCYGVSPTKLNDLCFTNVYADSFVIRGDEVRQIAPGQTGKIADYNYKLPDDFTGCVIAWNSNNLDSKVGGNYNYLYRLFRKSNLKPFERDISTEIYQAGSTPCNGVEGFNCYFPLQSYGFQPTNGVGYQPYRVVVLSFELLHAPATVCGPKKSTNLVKNKCVNFNFNGLTGTGVLTESNKKFLPFQQFGRDIADTTDAVRDPQTLEILDITPCSFGGVSVITPGTNTSNQVAVLYQDVNCTEVPVAIHADQLTPTWRVYSTGSNVFQTRAGCLIGAEHVNNSYECDIPIGAGICASYQTQTNSPRRAR

SEQ ID NO: 7 - DNA, 2016 bp, SARS-CoV-2
  misc_feature 1..2016: note = SARS-CoV-2 spike protein S1 subunit coding sequence
  source 1..2016: mol_type = other DNA
cagtgtgttaatcttacaaccagaactcaattaccccctgcatacactaattctttcacacgtggtgtttattaccctgacaaagttttcagatcctcagttttacattcaactcaggacttgttcttacctttcttttccaatgttacttggttccatgctatacatgtctctgggaccaatggtactaagaggtttgataaccctgtcctaccatttaatgatggtgtttattttgcttccactgagaagtctaacataataagaggctggatttttggtactactttagattcgaagacccagtccctacttattgttaataacgctactaatgttgttattaaagtctgtgaatttcaattttgtaatgatccatttttgggtgtttattaccacaaaaacaacaaaagttggatggaaagtgagttcagagtttattctagtgcgaataattgcacttttgaatatgtctctcagccttttcttatggaccttgaaggaaaacagggtaatttcaaaaatcttagggaatttgtgtttaagaatattgatggttattttaaaatatattctaagcacacgcctattaatttagtgcgtgatctccctcagggtttttcggctttagaaccattggtagatttgccaataggtattaacatcactaggtttcaaactttacttgctttacatagaagttatttgactcctggtgattcttcttcaggttggacagctggtgctgcagcttattatgtgggttatcttcaacctaggacttttctattaaaatataatgaaaatggaaccattacagatgctgtagactgtgcacttgaccctctctcagaaacaaagtgtacgttgaaatccttcactgtagaaaaaggaatctatcaaacttctaactttagagtccaaccaacagaatctattgttagatttcctaatattacaaacttgtgcccttttggtgaagtttttaacgccaccagatttgcatctgtttatgcttggaacaggaagagaatcagcaactgtgttgctgattattctgtcctatataattccgcatcattttccacttttaagtgttatggagtgtctcctactaaattaaatgatctctgctttactaatgtctatgcagattcatttgtaattagaggtgatgaagtcagacaaatcgctccagggcaaactggaaagattgctgattataattataaattaccagatgattttacaggctgcgttatagcttggaattctaacaatcttgattctaaggttggtggtaattataattacctgtatagattgtttaggaagtctaatctcaaaccttttgagagagatatttcaactgaaatctatcaggccggtagcacaccttgtaatggtgttgaaggttttaattgttactttcctttacaatcatatggtttccaacccactaatggtgttggttaccaaccatacagagtagtagtactttcttttgaacttctacatgcaccagcaactgtttgtggacctaaaaagtctactaatttggttaaaaacaaatgtgtcaatttcaacttcaatggtttaacaggcacaggtgttcttactgagtctaacaaaaagtttctgcctttccaacaatttggcagagacattgctgacactactgatgctgtccgtgatccacagacacttgagattcttgacattacaccatgttcttttggtggtgtcagtgttataacaccaggaacaaatacttctaaccaggttgctgttctttatcaggatgttaactgcacagaagtccctgttgctattcatgcagatcaacttactcctacttggcgtgtttattctacaggttctaatgtttttcaaacacgtgcaggctgtttaataggggctgaacatgtcaacaactcatatgagtgtgacatacccattggtgcaggtatatgcgctagttatcagactcagactaattctcctcggcgggcacgt

SEQ ID NO: 8 - protein, 223 aa, SARS-CoV-2
  REGION 1..223: note = SARS-CoV-2 spike protein receptor binding domain (RBD)spanning positions 319-541 (RBD-1)
RVQPTESIVRFPNITNLCPFGEVFNATRFASVYAWNRKRISNCVADYSVLYNSASFSTFKCYGVSPTKLNDLCFTNVYADSFVIRGDEVRQIAPGQTGKIADYNYKLPDDFTGCVIAWNSNNLDSKVGGNYNYLYRLFRKSNLKPFERDISTEIYQAGSTPCNGVEGFNCYFPLQSYGFQPTNGVGYQPYRVVVLSFELLHAPATVCGPKKSTNLVKNKCVNF

SEQ ID NO: 9 - DNA, 669 bp, SARS-CoV-2
  misc_feature 1..669: note = SARS-CoV-2 spike protein RBD-1 coding sequence
  source 1..669: mol_type = other DNA
agagtccaaccaacagaatctattgttagatttcctaatattacaaacttgtgcccttttggtgaagtttttaacgccaccagatttgcatctgtttatgcttggaacaggaagagaatcagcaactgtgttgctgattattctgtcctatataattccgcatcattttccacttttaagtgttatggagtgtctcctactaaattaaatgatctctgctttactaatgtctatgcagattcatttgtaattagaggtgatgaagtcagacaaatcgctccagggcaaactggaaagattgctgattataattataaattaccagatgattttacaggctgcgttatagcttggaactctaacaatcttgattctaaggttggtggtaattataattacctgtatagattgtttaggaagtctaatctcaaaccttttgagagagatatttcaactgaaatctatcaggccggtagcacaccttgtaatggtgttgaaggttttaattgttactttcctttacaatcatatggtttccaacccactaatggtgttggttaccaaccatacagagtagtagtactttcttttgaacttctacatgcaccagcaactgtttgtggacctaaaaagtctactaatttggttaaaaacaaatgtgtcaatttc

SEQ ID NO: 10 - protein, 199 aa, SARS-CoV-2
  REGION 1..199: note = SARS-CoV-2 spike protein RBD spanning positions 331-529 (RBD-2)
NITNLCPFGEVFNATRFASVYAWNRKRISNCVADYSVLYNSASFSTFKCYGVSPTKLNDLCFTNVYADSFVIRGDEVRQIAPGQTGKIADYNYKLPDDFTGCVIAWNSNNLDSKVGGNYNYLYRLFRKSNLKPFERDISTEIYQAGSTPCNGVEGFNCYFPLQSYGFQPTNGVGYQPYRVVVLSFELLHAPATVCGPKK

SEQ ID NO: 11 - DNA, 597 bp, SARS-CoV-2
  misc_feature 1..597: note = SARS-CoV-2 spike protein RBD-2 coding sequence
  source 1..597: mol_type = other DNA
aatattacaaacttgtgcccttttggtgaagtttttaacgccaccagatttgcatctgtttatgcttggaacaggaagagaatcagcaactgtgttgctgattattctgtcctatataattccgcatcattttccacttttaagtgttatggagtgtctcctactaaattaaatgatctctgctttactaatgtctatgcagattcatttgtaattagaggtgatgaagtcagacaaatcgctccagggcaaactggaaagattgctgattataattataaattaccagatgattttacaggctgcgttatagcttggaactctaacaatcttgattctaaggttggtggtaattataattacctgtatagattgtttaggaagtctaatctcaaaccttttgagagagatatttcaactgaaatctatcaggccggtagcacaccttgtaatggtgttgaaggttttaattgttactttcctttacaatcatatggtttccaacccactaatggtgttggttaccaaccatacagagtagtagtactttcttttgaacttctacatgcaccagcaactgtttgtggacctaaaaag

SEQ ID NO: 12 - protein, 194 aa, SARS-CoV-2
  REGION 1..194: note = SARS-CoV-2 spike protein RBD spanning positions 331-524 (RBD-3)
NITNLCPFGEVFNATRFASVYAWNRKRISNCVADYSVLYNSASFSTFKCYGVSPTKLNDLCFTNVYADSFVIRGDEVRQIAPGQTGKIADYNYKLPDDFTGCVIAWNSNNLDSKVGGNYNYLYRLFRKSNLKPFERDISTEIYQAGSTPCNGVEGFNCYFPLQSYGFQPTNGVGYQPYRVVVLSFELLHAPATV

SEQ ID NO: 13 - DNA, 582 bp, SARS-CoV-2
  misc_feature 1..582: note = SARS-CoV-2 spike protein RBD-3 coding sequence
  source 1..582: mol_type = other DNA
aatattacaaacttgtgcccttttggtgaagtttttaacgccaccagatttgcatctgtttatgcttggaacaggaagagaatcagcaactgtgttgctgattattctgtcctatataattccgcatcattttccacttttaagtgttatggagtgtctcctactaaattaaatgatctctgctttactaatgtctatgcagattcatttgtaattagaggtgatgaagtcagacaaatcgctccagggcaaactggaaagattgctgattataattataaattaccagatgattttacaggctgcgttatagcttggaactctaacaatcttgattctaaggttggtggtaattataattacctgtatagattgtttaggaagtctaatctcaaaccttttgagagagatatttcaactgaaatctatcaggccggtagcacaccttgtaatggtgttgaaggttttaattgttactttcctttacaatcatatggtttccaacccactaatggtgttggttaccaaccatacagagtagtagtactttcttttgaacttctacatgcaccagcaactgtt

SEQ ID NO: 14 - protein, 211 aa, SARS-CoV-2
  REGION 1..211: note = SARS-CoV-2 spike protein RBD spanning positions 319-529 (RBD-4)
RVQPTESIVRFPNITNLCPFGEVFNATRFASVYAWNRKRISNCVADYSVLYNSASFSTFKCYGVSPTKLNDLCFTNVYADSFVIRGDEVRQIAPGQTGKIADYNYKLPDDFTGCVIAWNSNNLDSKVGGNYNYLYRLFRKSNLKPFERDISTEIYQAGSTPCNGVEGFNCYFPLQSYGFQPTNGVGYQPYRVVVLSFELLHAPATVCGPKK

SEQ ID NO: 15 - DNA, 633 bp, SARS-CoV-2
  misc_feature 1..633: note = SARS-CoV-2 spike protein RBD-4 coding sequence
  source 1..633: mol_type = other DNA
agagtccaaccaacagaatctattgttagatttcctaatattacaaacttgtgcccttttggtgaagtttttaacgccaccagatttgcatctgtttatgcttggaacaggaagagaatcagcaactgtgttgctgattattctgtcctatataattccgcatcattttccacttttaagtgttatggagtgtctcctactaaattaaatgatctctgctttactaatgtctatgcagattcatttgtaattagaggtgatgaagtcagacaaatcgctccagggcaaactggaaagattgctgattataattataaattaccagatgattttacaggctgcgttatagcttggaactctaacaatcttgattctaaggttggtggtaattataattacctgtatagattgtttaggaagtctaatctcaaaccttttgagagagatatttcaactgaaatctatcaggccggtagcacaccttgtaatggtgttgaaggttttaattgttactttcctttacaatcatatggtttccaacccactaatggtgttggttaccaaccatacagagtagtagtactttcttttgaacttctacatgcaccagcaactgtttgtggacctaaaaag

SEQ ID NO: 16 - protein, 56 aa, SARS-CoV-2
  REGION 1..56: note = SARS-CoV-2 spike protein receptor binding motif (RBM)
VGGNYNYLYRLFRKSNLKPFERDISTEIYQAGSTPCNGVEGFNCYFPLQSYGFQPT

SEQ ID NO: 17 - DNA, 168 bp, SARS-CoV-2
  misc_feature 1..168: note = SARS-CoV-2 spike protein RBM coding sequence
  source 1..168: mol_type = other DNA
gttggtggtaattataattacctgtatagattgtttaggaagtctaatctcaaaccttttgagagagatatttcaactgaaatctatcaggccggtagcacaccttgtaatggtgttgaaggttttaattgttactttcctttacaatcatatggtttccaacccact

SEQ ID NO: 18 - protein, 419 aa, SARS-CoV-2
  REGION 1..419: note = SARS-CoV-2 nucleocapsid protein
MSDNGPQNQRNAPRITFGGPSDSTGSNQNGERSGARSKQRRPQGLPNNTASWFTALTQHGKEDLKFPRGQGVPINTNSSPDDQIGYYRRATRRIRGGDGKMKDLSPRWYFYYLGTGPEAGLPYGANKDGIIWVATEGALNTPKDHIGTRNPANNAAIVLQLPQGTTLPKGFYAEGSRGGSQASSRSSSRSRNSSRNSTPGSSRGTSPARMAGNGGDAALALLLLDRLNQLESKMSGKGQQQQGQTVTKKSAAEASKKPRQKRTATKAYNVTQAFGRRGPEQTQGNFGDQELIRQGTDYKHWPQIAQFAPSASAFFGMSRIGMEVTPSGTWLTYTAAIKLDDKDPNFKDQVILLNKHIDAYKTFPPTEPKKDKKKKADETQALPQRQKKQQTVTLLPAADLDDFSKQLQQSMSSADSTQA

SEQ ID NO: 19 - DNA, 1257 bp, SARS-CoV-2
  misc_feature 1..1257: note = SARS-CoV-2 nucleocapsid protein coding sequence
  source 1..1257: mol_type = other DNA
atgtctgataatggaccccaaaatcagcgaaatgcaccccgcattacgtttggtggaccctcagattcaactggcagtaaccagaatggagaacgcagtggggcgcgatcaaaacaacgtcggccccaaggtttacccaataatactgcgtcttggttcaccgctctcactcaacatggcaaggaagaccttaaattccctcgaggacaaggcgttccaattaacaccaatagcagtccagatgaccaaattggctactaccgaagagctaccagacgaattcgtggtggtgacggtaaaatgaaagatctcagtccaagatggtatttctactacctaggaactgggccagaagctggacttccctatggtgctaacaaagacggcatcatatgggttgcaactgagggagccttgaatacaccaaaagatcacattggcacccgcaatcctgctaacaatgctgcaatcgtgctacaacttcctcaaggaacaacattgccaaaaggcttctacgcagaagggagcagaggcggcagtcaagcctcttctcgttcctcatcacgtagtcgcaacagttcaagaaattcaactccaggcagcagtaggggaacttctcctgctagaatggctggcaatggcggtgatgctgctcttgctttgctgctgcttgacagattgaaccagcttgagagcaaaatgtctggtaaaggccaacaacaacaaggccaaactgtcactaagaaatctgctgctgaggcttctaagaagcctcggcaaaaacgtactgccactaaagcatacaatgtaacacaagctttcggcagacgtggtccagaacaaacccaaggaaattttggggaccaggaactaatcagacaaggaactgattacaaacattggccgcaaattgcacaatttgcccccagcgcttcagcgttcttcggaatgtcgcgcattggcatggaagtcacaccttcgggaacgtggttgacctacacagctgccatcaaattggatgacaaagatccaaatttcaaagatcaagtcattttgctgaataagcatattgacgcatacaaaacattcccaccaacagagcctaaaaaggacaaaaagaagaaggctgatgaaactcaagccttaccgcagagacagaagaaacagcaaactgtgactcttcttcctgctgcagatttggatgatttctccaaacaattgcaacaatccatgagcagtgctgactcaactcaggcc

SEQ ID NO: 20 - protein, 1273 aa, synthetic construct
  REGION 1..1273: note = SARS-CoV-2 spike protein with native signal peptide andan N501T substitution
MFVFLVLLPLVSSQCVNLTTRTQLPPAYTNSFTRGVYYPDKVFRSSVLHSTQDLFLPFFSNVTWFHAIHVSGTNGTKRFDNPVLPFNDGVYFASTEKSNIIRGWIFGTTLDSKTQSLLIVNNATNVVIKVCEFQFCNDPFLGVYYHKNNKSWMESEFRVYSSANNCTFEYVSQPFLMDLEGKQGNFKNLREFVFKNIDGYFKIYSKHTPINLVRDLPQGFSALEPLVDLPIGINITRFQTLLALHRSYLTPGDSSSGWTAGAAAYYVGYLQPRTFLLKYNENGTITDAVDCALDPLSETKCTLKSFTVEKGIYQTSNFRVQPTESIVRFPNITNLCPFGEVFNATRFASVYAWNRKRISNCVADYSVLYNSASFSTFKCYGVSPTKLNDLCFTNVYADSFVIRGDEVRQIAPGQTGKIADYNYKLPDDFTGCVIAWNSNNLDSKVGGNYNYLYRLFRKSNLKPFERDISTEIYQAGSTPCNGVEGFNCYFPLQSYGFQPTTGVGYQPYRVVVLSFELLHAPATVCGPKKSTNLVKNKCVNFNFNGLTGTGVLTESNKKFLPFQQFGRDIADTTDAVRDPQTLEILDITPCSFGGVSVITPGTNTSNQVAVLYQDVNCTEVPVAIHADQLTPTWRVYSTGSNVFQTRAGCLIGAEHVNNSYECDIPIGAGICASYQTQTNSPRRARSVASQSIIAYTMSLGAENSVAYSNNSIAIPTNFTISVTTEILPVSMTKTSVDCTMYICGDSTECSNLLLQYGSFCTQLNRALTGIAVEQDKNTQEVFAQVKQIYKTPPIKDFGGFNFSQILPDPSKPSKRSFIEDLLFNKVTLADAGFIKQYGDCLGDIAARDLICAQKFNGLTVLPPLLTDEMIAQYTSALLAGTITSGWTFGAGAALQIPFAMQMAYRFNGIGVTQNVLYENQKLIANQFNSAIGKIQDSLSSTASALGKLQDVVNQNAQALNTLVKQLSSNFGAISSVLNDILSRLDKVEAEVQIDRLITGRLQSLQTYVTQQLIRAAEIRASANLAATKMSECVLGQSKRVDFCGKGYHLMSFPQSAPHGVVFLHVTYVPAQEKNFTTAPAICHDGKAHFPREGVFVSNGTHWFVTQRNFYEPQIITTDNTFVSGNCDVVIGIVNNTVYDPLQPELDSFKEELDKYFKNHTSPDVDLGDISGINASVVNIQKEIDRLNEVAKNLNESLIDLQELGKYEQYIKWPWYIWLGFIAGLIAIVMVTIMLCCMTSCCSCLKGCCSCGSCCKFDEDDSEPVLKGVKLHYT

SEQ ID NO: 21 - protein, 1198 aa, synthetic construct
  REGION 1..1198: note = SARS-CoV-2 spike protein ECD with an N501T substitution
QCVNLTTRTQLPPAYTNSFTRGVYYPDKVFRSSVLHSTQDLFLPFFSNVTWFHAIHVSGTNGTKRFDNPVLPFNDGVYFASTEKSNIIRGWIFGTTLDSKTQSLLIVNNATNVVIKVCEFQFCNDPFLGVYYHKNNKSWMESEFRVYSSANNCTFEYVSQPFLMDLEGKQGNFKNLREFVFKNIDGYFKIYSKHTPINLVRDLPQGFSALEPLVDLPIGINITRFQTLLALHRSYLTPGDSSSGWTAGAAAYYVGYLQPRTFLLKYNENGTITDAVDCALDPLSETKCTLKSFTVEKGIYQTSNFRVQPTESIVRFPNITNLCPFGEVFNATRFASVYAWNRKRISNCVADYSVLYNSASFSTFKCYGVSPTKLNDLCFTNVYADSFVIRGDEVRQIAPGQTGKIADYNYKLPDDFTGCVIAWNSNNLDSKVGGNYNYLYRLFRKSNLKPFERDISTEIYQAGSTPCNGVEGFNCYFPLQSYGFQPTTGVGYQPYRVVVLSFELLHAPATVCGPKKSTNLVKNKCVNFNFNGLTGTGVLTESNKKFLPFQQFGRDIADTTDAVRDPQTLEILDITPCSFGGVSVITPGTNTSNQVAVLYQDVNCTEVPVAIHADQLTPTWRVYSTGSNVFQTRAGCLIGAEHVNNSYECDIPIGAGICASYQTQTNSPRRARSVASQSIIAYTMSLGAENSVAYSNNSIAIPTNFTISVTTEILPVSMTKTSVDCTMYICGDSTECSNLLLQYGSFCTQLNRALTGIAVEQDKNTQEVFAQVKQIYKTPPIKDFGGFNFSQILPDPSKPSKRSFIEDLLFNKVTLADAGFIKQYGDCLGDIAARDLICAQKFNGLTVLPPLLTDEMIAQYTSALLAGTITSGWTFGAGAALQIPFAMQMAYRFNGIGVTQNVLYENQKLIANQFNSAIGKIQDSLSSTASALGKLQDVVNQNAQALNTLVKQLSSNFGAISSVLNDILSRLDKVEAEVQIDRLITGRLQSLQTYVTQQLIRAAEIRASANLAATKMSECVLGQSKRVDFCGKGYHLMSFPQSAPHGVVFLHVTYVPAQEKNFTTAPAICHDGKAHFPREGVFVSNGTHWFVTQRNFYEPQIITTDNTFVSGNCDVVIGIVNNTVYDPLQPELDSFKEELDKYFKNHTSPDVDLGDISGINASVVNIQKEIDRLNEVAKNLNESLIDLQELGKYEQYIK

SEQ ID NO: 22 - protein, 672 aa, synthetic construct
  REGION 1..672: note = SARS-CoV-2 spike protein S1 subunit with an N501T substitution
QCVNLTTRTQLPPAYTNSFTRGVYYPDKVFRSSVLHSTQDLFLPFFSNVTWFHAIHVSGTNGTKRFDNPVLPFNDGVYFASTEKSNIIRGWIFGTTLDSKTQSLLIVNNATNVVIKVCEFQFCNDPFLGVYYHKNNKSWMESEFRVYSSANNCTFEYVSQPFLMDLEGKQGNFKNLREFVFKNIDGYFKIYSKHTPINLVRDLPQGFSALEPLVDLPIGINITRFQTLLALHRSYLTPGDSSSGWTAGAAAYYVGYLQPRTFLLKYNENGTITDAVDCALDPLSETKCTLKSFTVEKGIYQTSNFRVQPTESIVRFPNITNLCPFGEVFNATRFASVYAWNRKRISNCVADYSVLYNSASFSTFKCYGVSPTKLNDLCFTNVYADSFVIRGDEVRQIAPGQTGKIADYNYKLPDDFTGCVIAWNSNNLDSKVGGNYNYLYRLFRKSNLKPFERDISTEIYQAGSTPCNGVEGFNCYFPLQSYGFQPTTGVGYQPYRVVVLSFELLHAPATVCGPKKSTNLVKNKCVNFNFNGLTGTGVLTESNKKFLPFQQFGRDIADTTDAVRDPQTLEILDITPCSFGGVSVITPGTNTSNQVAVLYQDVNCTEVPVAIHADQLTPTWRVYSTGSNVFQTRAGCLIGAEHVNNSYECDIPIGAGICASYQTQTNSPRRAR

SEQ ID NO: 23 - protein, 223 aa, synthetic construct
  REGION 1..223: note = SARS-CoV-2 spike protein RBD-1 with an N501T substitution
RVQPTESIVRFPNITNLCPFGEVFNATRFASVYAWNRKRISNCVADYSVLYNSASFSTFKCYGVSPTKLNDLCFTNVYADSFVIRGDEVRQIAPGQTGKIADYNYKLPDDFTGCVIAWNSNNLDSKVGGNYNYLYRLFRKSNLKPFERDISTEIYQAGSTPCNGVEGFNCYFPLQSYGFQPTTGVGYQPYRVVVLSFELLHAPATVCGPKKSTNLVKNKCVNF

SEQ ID NO: 24 - protein, 198 aa, synthetic construct
  REGION 1..198: note = SARS-CoV-2 spike protein RBD-2 with an N501Tsubstitution (RBD-6)
ITNLCPFGEVFNATRFASVYAWNRKRISNCVADYSVLYNSASFSTFKCYGVSPTKLNDLCFTNVYADSFVIRGDEVRQIAPGQTGKIADYNYKLPDDFTGCVIAWNSNNLDSKVGGNYNYLYRLFRKSNLKPFERDISTEIYQAGSTPCNGVEGFNCYFPLQSYGFQPTTGVGYQPYRVVVLSFELLHAPATVCGPKK

SEQ ID NO: 25 - protein, 194 aa, synthetic construct
  REGION 1..194: note = SARS-CoV-2 spike protein RBD-3 with an N501Tsubstitution (RBD-7)
NITNLCPFGEVFNATRFASVYAWNRKRISNCVADYSVLYNSASFSTFKCYGVSPTKLNDLCFTNVYADSFVIRGDEVRQIAPGQTGKIADYNYKLPDDFTGCVIAWNSNNLDSKVGGNYNYLYRLFRKSNLKPFERDISTEIYQAGSTPCNGVEGFNCYFPLQSYGFQPTTGVGYQPYRVVVLSFELLHAPATV

SEQ ID NO: 26 - protein, 211 aa, synthetic construct
  REGION 1..211: note = SARS-CoV-2 spike protein RBD-4 with an N501Tsubstitution (RBD-8)
RVQPTESIVRFPNITNLCPFGEVFNATRFASVYAWNRKRISNCVADYSVLYNSASFSTFKCYGVSPTKLNDLCFTNVYADSFVIRGDEVRQIAPGQTGKIADYNYKLPDDFTGCVIAWNSNNLDSKVGGNYNYLYRLFRKSNLKPFERDISTEIYQAGSTPCNGVEGFNCYFPLQSYGFQPTTGVGYQPYRVVVLSFELLHAPATVCGPKK

SEQ ID NO: 27 - DNA, 633 bp, synthetic construct
  misc_feature 1..633: note = SARS-CoV-2 spike protein RBD-8 coding sequence
  source 1..633: mol_type = other DNA
agagtccaaccaacagaatctattgttagatttcctaatattacaaacttgtgcccttttggtgaagtttttaacgccaccagatttgcatctgtttatgcttggaacaggaagagaatcagcaactgtgttgctgattattctgtcctatataattccgcatcattttccacttttaagtgttatggagtgtctcctactaaattaaatgatctctgctttactaatgtctatgcagattcatttgtaattagaggtgatgaagtcagacaaatcgctccagggcaaactggaaagattgctgattataattataaattaccagatgattttacaggctgcgttatagcttggaactctaacaatcttgattctaaggttggtggtaattataattacctgtatagattgtttaggaagtctaatctcaaaccttttgagagagatatttcaactgaaatctatcaggccggtagcacaccttgtaatggtgttgaaggttttaattgttactttcctttacaatcatatggtttccaacccactactggtgttggttaccaaccatacagagtagtagtactttcttttgaacttctacatgcaccagcaactgtttgtggacctaaaaag

SEQ ID NO: 28 - protein, 8 aa, synthetic construct
  REGION 1..8: note = (G3S)2 linker peptide
GGGSGGGS

SEQ ID NO: 29 - DNA, 24 bp, synthetic construct
  misc_feature 1..24: note = (G3S)2 linker peptide coding sequence
  source 1..24: mol_type = other DNA
ggaggaggaagtggaggaggaagt

SEQ ID NO: 30 - protein, 28 aa, synthetic construct
  REGION 1..28: note = Trimmerization peptide
GYIPEAPRDGQAYVRKDGEWVLLSTFLG

SEQ ID NO: 31 - DNA, 84 bp, synthetic construct
  misc_feature 1..84: note = Trimmerization peptide coding sequence
  source 1..84: mol_type = other DNA
ggctatattccggaagcgccgcgcgatggccaggcgtatgtgcgcaaagatggcgaatgggtgctgctgagcacctttctgggc

SEQ ID NO: 32 - protein, 1234 aa, synthetic construct
  REGION 1..1234: note = SARS-CoV-2 spike protein ECD with C terminal fusion of a(G3S)2 linker and a trimmerization peptide
QCVNLTTRTQLPPAYTNSFTRGVYYPDKVFRSSVLHSTQDLFLPFFSNVTWFHAIHVSGTNGTKRFDNPVLPFNDGVYFASTEKSNIIRGWIFGTTLDSKTQSLLIVNNATNVVIKVCEFQFCNDPFLGVYYHKNNKSWMESEFRVYSSANNCTFEYVSQPFLMDLEGKQGNFKNLREFVFKNIDGYFKIYSKHTPINLVRDLPQGFSALEPLVDLPIGINITRFQTLLALHRSYLTPGDSSSGWTAGAAAYYVGYLQPRTFLLKYNENGTITDAVDCALDPLSETKCTLKSFTVEKGIYQTSNFRVQPTESIVRFPNITNLCPFGEVFNATRFASVYAWNRKRISNCVADYSVLYNSASFSTFKCYGVSPTKLNDLCFTNVYADSFVIRGDEVRQIAPGQTGKIADYNYKLPDDFTGCVIAWNSNNLDSKVGGNYNYLYRLFRKSNLKPFERDISTEIYQAGSTPCNGVEGFNCYFPLQSYGFQPTNGVGYQPYRVVVLSFELLHAPATVCGPKKSTNLVKNKCVNFNFNGLTGTGVLTESNKKFLPFQQFGRDIADTTDAVRDPQTLEILDITPCSFGGVSVITPGTNTSNQVAVLYQDVNCTEVPVAIHADQLTPTWRVYSTGSNVFQTRAGCLIGAEHVNNSYECDIPIGAGICASYQTQTNSPRRARSVASQSIIAYTMSLGAENSVAYSNNSIAIPTNFTISVTTEILPVSMTKTSVDCTMYICGDSTECSNLLLQYGSFCTQLNRALTGIAVEQDKNTQEVFAQVKQIYKTPPIKDFGGFNFSQILPDPSKPSKRSFIEDLLFNKVTLADAGFIKQYGDCLGDIAARDLICAQKFNGLTVLPPLLTDEMIAQYTSALLAGTITSGWTFGAGAALQIPFAMQMAYRFNGIGVTQNVLYENQKLIANQFNSAIGKIQDSLSSTASALGKLQDVVNQNAQALNTLVKQLSSNFGAISSVLNDILSRLDKVEAEVQIDRLITGRLQSLQTYVTQQLIRAAEIRASANLAATKMSECVLGQSKRVDFCGKGYHLMSFPQSAPHGVVFLHVTYVPAQEKNFTTAPAICHDGKAHFPREGVFVSNGTHWFVTQRNFYEPQIITTDNTFVSGNCDVVIGIVNNTVYDPLQPELDSFKEELDKYFKNHTSPDVDLGDISGINASVVNIQKEIDRLNEVAKNLNESLIDLQELGKYEQYIKGGGSGGGSGYIPEAPRDGQAYVRKDGEWVLLSTFLG

SEQ ID NO: 33 - DNA, 3702 bp, synthetic construct
  misc_feature 1..3702: note = SARS-CoV-2 spike protein ECD with C terminal fusion of a(G3S)2 linker and a trimmerization peptide coding sequence
  source 1..3702: mol_type = other DNA
cagtgtgttaatcttacaaccagaactcaattaccccctgcatacactaattctttcacacgtggtgtttattaccctgacaaagttttcagatcctcagttttacattcaactcaggacttgttcttacctttcttttccaatgttacttggttccatgctatacatgtctctgggaccaatggtactaagaggtttgataaccctgtcctaccatttaatgatggtgtttattttgcttccactgagaagtctaacataataagaggctggatttttggtactactttagattcgaagacccagtccctacttattgttaataacgctactaatgttgttattaaagtctgtgaatttcaattttgtaatgatccatttttgggtgtttattaccacaaaaacaacaaaagttggatggaaagtgagttcagagtttattctagtgcgaataattgcacttttgaatatgtctctcagccttttcttatggaccttgaaggaaaacagggtaatttcaaaaatcttagggaatttgtgtttaagaatattgatggttattttaaaatatattctaagcacacgcctattaatttagtgcgtgatctccctcagggtttttcggctttagaaccattggtagatttgccaataggtattaacatcactaggtttcaaactttacttgctttacatagaagttatttgactcctggtgattcttcttcaggttggacagctggtgctgcagcttattatgtgggttatcttcaacctaggacttttctattaaaatataatgaaaatggaaccattacagatgctgtagactgtgcacttgaccctctctcagaaacaaagtgtacgttgaaatccttcactgtagaaaaaggaatctatcaaacttctaactttagagtccaaccaacagaatctattgttagatttcctaatattacaaacttgtgcccttttggtgaagtttttaacgccaccagatttgcatctgtttatgcttggaacaggaagagaatcagcaactgtgttgctgattattctgtcctatataattccgcatcattttccacttttaagtgttatggagtgtctcctactaaattaaatgatctctgctttactaatgtctatgcagattcatttgtaattagaggtgatgaagtcagacaaatcgctccagggcaaactggaaagattgctgattataattataaattaccagatgattttacaggctgcgttatagcttggaactctaacaatcttgattctaaggttggtggtaattataattacctgtatagattgtttaggaagtctaatctcaaaccttttgagagagatatttcaactgaaatctatcaggccggtagcacaccttgtaatggtgttgaaggttttaattgttactttcctttacaatcatatggtttccaacccactaatggtgttggttaccaaccatacagagtagtagtactttcttttgaacttctacatgcaccagcaactgtttgtggacctaaaaagtctactaatttggttaaaaacaaatgtgtcaatttcaacttcaatggtttaacaggcacaggtgttcttactgagtctaacaaaaagtttctgcctttccaacaatttggcagagacattgctgacactactgatgctgtccgtgatccacagacacttgagattcttgacattacaccatgttcttttggtggtgtcagtgttataacaccaggaacaaatacttctaaccaggttgctgttctttatcaggatgttaactgcacagaagtccctgttgctattcatgcagatcaacttactcctacttggcgtgtttattctacaggttctaatgtttttcaaacacgtgcaggctgtttaataggggctgaacatgtcaacaactcatatgagtgtgacatacccattggtgcaggtatatgcgctagttatcagactcagactaattctcctcggcgggcacgtagtgtagctagtcaatccatcattgcctacactatgtcacttggtgcagaaaattcagttgcttactctaataactctattgccatacccacaaattttactattagtgttaccacagaaattctaccagtgtctatgaccaagacatcagtagattgtacaatgtacatttgtggtgattcaactgaatgcagcaatcttttgttgcaatatggcagtttttgtacacaattaaaccgtgctttaactggaatagctgttgaacaagacaaaaacacccaagaagtttttgcacaagtcaaacaaatttacaaaacaccaccaattaaagattttggtggttttaatttttcacaaatattaccagatccatcaaaaccaagcaagaggtcatttattgaagatctacttttcaacaaagtgacacttgcagatgctggcttcatcaaacaatatggtgattgccttggtgatattgctgctagagacctcatttgtgcacaaaagtttaacggccttactgttttgccacctttgctcacagatgaaatgattgctcaatacacttctgcactgttagcgggtacaatcacttctggttggacctttggtgcaggtgctgcattacaaataccatttgctatgcaaatggcttataggtttaatggtattggagttacacagaatgttctctatgagaaccaaaaattgattgccaaccaatttaatagtgctattggcaaaattcaagactcactttcttccacagcaagtgcacttggaaaacttcaagatgtggtcaaccaaaatgcacaagctttaaacacgcttgttaaacaacttagctccaattttggtgcaatttcaagtgttttaaatgatatcctttcacgtcttgacaaagttgaggctgaagtgcaaattgataggttgatcacaggcagacttcaaagtttgcagacatatgtgactcaacaattaattagagctgcagaaatcagagcttctgctaatcttgctgctactaaaatgtcagagtgtgtacttggacaatcaaaaagagttgatttttgtggaaagggctatcatcttatgtccttccctcagtcagcacctcatggtgtagtcttcttgcatgtgacttatgtccctgcacaagaaaagaacttcacaactgctcctgccatttgtcatgatggaaaagcacactttcctcgtgaaggtgtctttgtttcaaatggcacacactggtttgtaacacaaaggaatttttatgaaccacaaatcattactacagacaacacatttgtgtctggtaactgtgatgttgtaataggaattgtcaacaacacagtttatgatcctttgcaacctgaattagactcattcaaggaggagttagataaatattttaagaatcatacatcaccagatgttgatttaggtgacatctctggcattaatgcttcagttgtaaacattcaaaaagaaattgaccgcctcaatgaggttgccaagaatttaaatgaatctctcatcgatctccaagaacttggaaagtatgagcagtatataaaaggaggaggaagtggaggaggaagtggctatattccggaagcgccgcgcgatggccaggcgtatgtgcgcaaagatggcgaatgggtgctgctgagcacctttctgggc

SEQ ID NO: 34 - protein, 235 aa, synthetic construct
  REGION 1..235: note = SARS-CoV-2 spike protein RBD-2 with C-terminal fusion of a(G3S)2 linker and a trimmerization peptide
NITNLCPFGEVFNATRFASVYAWNRKRISNCVADYSVLYNSASFSTFKCYGVSPTKLNDLCFTNVYADSFVIRGDEVRQIAPGQTGKIADYNYKLPDDFTGCVIAWNSNNLDSKVGGNYNYLYRLFRKSNLKPFERDISTEIYQAGSTPCNGVEGFNCYFPLQSYGFQPTNGVGYQPYRVVVLSFELLHAPATVCGPKKGGGSGGGSGYIPEAPRDGQAYVRKDGEWVLLSTFLG

SEQ ID NO: 35 - DNA, 705 bp, synthetic construct
  misc_feature 1..705: note = SARS-CoV-2 spike protein RBD-2 with C-terminal fusion of a(G3S)2 linker and a trimmerization peptide coding sequence
  source 1..705: mol_type = other DNA
aatattacaaacttgtgcccttttggtgaagtttttaacgccaccagatttgcatctgtttatgcttggaacaggaagagaatcagcaactgtgttgctgattattctgtcctatataattccgcatcattttccacttttaagtgttatggagtgtctcctactaaattaaatgatctctgctttactaatgtctatgcagattcatttgtaattagaggtgatgaagtcagacaaatcgctccagggcaaactggaaagattgctgattataattataaattaccagatgattttacaggctgcgttatagcttggaactctaacaatcttgattctaaggttggtggtaattataattacctgtatagattgtttaggaagtctaatctcaaaccttttgagagagatatttcaactgaaatctatcaggccggtagcacaccttgtaatggtgttgaaggttttaattgttactttcctttacaatcatatggtttccaacccactaatggtgttggttaccaaccatacagagtagtagtactttcttttgaacttctacatgcaccagcaactgtttgtggacctaaaaagggaggaggaagtggaggaggaagtggctatattccggaagcgccgcgcgatggccaggcgtatgtgcgcaaagatggcgaatgggtgctgctgagcacctttctgggc

SEQ ID NO: 36 - protein, 13 aa, synthetic construct
  REGION 1..13: note = SARS-CoV-2 spike protein native signal peptide
MFVFLVLLPLVSS

SEQ ID NO: 37 - DNA, 39 bp, SARS-CoV-2
  misc_feature 1..39: note = SARS-CoV-2 spike protein native signal peptide coding sequence
  source 1..39: mol_type = other DNA
atgtttgtttttcttgttttattgccattagtctctagt

SEQ ID NO: 38 - protein, 18 aa, synthetic construct
  REGION 1..18: note = Human IgE signal peptide
MDWTWILFLVAAATRVHS

SEQ ID NO: 39 - DNA, 54 bp, synthetic construct
  misc_feature 1..54: note = Human IgE signal peptide coding sequence
  source 1..54: mol_type = other DNA
atggactggacctggattctcttcttggtggcagcagccacgcgagtccactcc

SEQ ID NO: 40 - protein, 1260 aa, synthetic construct
  REGION 1..1260: note = SARS-CoV-2 spike protein without native signal peptide
QCVNLTTRTQLPPAYTNSFTRGVYYPDKVFRSSVLHSTQDLFLPFFSNVTWFHAIHVSGTNGTKRFDNPVLPFNDGVYFASTEKSNIIRGWIFGTTLDSKTQSLLIVNNATNVVIKVCEFQFCNDPFLGVYYHKNNKSWMESEFRVYSSANNCTFEYVSQPFLMDLEGKQGNFKNLREFVFKNIDGYFKIYSKHTPINLVRDLPQGFSALEPLVDLPIGINITRFQTLLALHRSYLTPGDSSSGWTAGAAAYYVGYLQPRTFLLKYNENGTITDAVDCALDPLSETKCTLKSFTVEKGIYQTSNFRVQPTESIVRFPNITNLCPFGEVFNATRFASVYAWNRKRISNCVADYSVLYNSASFSTFKCYGVSPTKLNDLCFTNVYADSFVIRGDEVRQIAPGQTGKIADYNYKLPDDFTGCVIAWNSNNLDSKVGGNYNYLYRLFRKSNLKPFERDISTEIYQAGSTPCNGVEGFNCYFPLQSYGFQPTNGVGYQPYRVVVLSFELLHAPATVCGPKKSTNLVKNKCVNFNFNGLTGTGVLTESNKKFLPFQQFGRDIADTTDAVRDPQTLEILDITPCSFGGVSVITPGTNTSNQVAVLYQDVNCTEVPVAIHADQLTPTWRVYSTGSNVFQTRAGCLIGAEHVNNSYECDIPIGAGICASYQTQTNSPRRARSVASQSIIAYTMSLGAENSVAYSNNSIAIPTNFTISVTTEILPVSMTKTSVDCTMYICGDSTECSNLLLQYGSFCTQLNRALTGIAVEQDKNTQEVFAQVKQIYKTPPIKDFGGFNFSQILPDPSKPSKRSFIEDLLFNKVTLADAGFIKQYGDCLGDIAARDLICAQKFNGLTVLPPLLTDEMIAQYTSALLAGTITSGWTFGAGAALQIPFAMQMAYRFNGIGVTQNVLYENQKLIANQFNSAIGKIQDSLSSTASALGKLQDVVNQNAQALNTLVKQLSSNFGAISSVLNDILSRLDKVEAEVQIDRLITGRLQSLQTYVTQQLIRAAEIRASANLAATKMSECVLGQSKRVDFCGKGYHLMSFPQSAPHGVVFLHVTYVPAQEKNFTTAPAICHDGKAHFPREGVFVSNGTHWFVTQRNFYEPQIITTDNTFVSGNCDVVIGIVNNTVYDPLQPELDSFKEELDKYFKNHTSPDVDLGDISGINASVVNIQKEIDRLNEVAKNLNESLIDLQELGKYEQYIKWPWYIWLGFIAGLIAIVMVTIMLCCMTSCCSCLKGCCSCGSCCKFDEDDSEPVLKGVKLHYT

SEQ ID NO: 41 - DNA, 3633 bp, synthetic construct
  misc_feature 1..3633: note = SARS-CoV-2 spike protein without native signal peptidecoding sequence
  source 1..3633: mol_type = other DNA
atgtttgtttttcttgttttattgccattagtctctagtcagtgtgttaatcttacaaccagaactcaattaccccctgcatacactaattctttcacacgtggtgtttattaccctgacaaagttttcagatcctcagttttacattcaactcaggacttgttcttacctttcttttccaatgttacttggttccatgctatacatgtctctgggaccaatggtactaagaggtttgataaccctgtcctaccatttaatgatggtgtttattttgcttccactgagaagtctaacataataagaggctggatttttggtactactttagattcgaagacccagtccctacttattgttaataacgctactaatgttgttattaaagtctgtgaatttcaattttgtaatgatccatttttgggtgtttattaccacaaaaacaacaaaagttggatggaaagtgagttcagagtttattctagtgcgaataattgcacttttgaatatgtctctcagccttttcttatggaccttgaaggaaaacagggtaatttcaaaaatcttagggaatttgtgtttaagaatattgatggttattttaaaatatattctaagcacacgcctattaatttagtgcgtgatctccctcagggtttttcggctttagaaccattggtagatttgccaataggtattaacatcactaggtttcaaactttacttgctttacatagaagttatttgactcctggtgattcttcttcaggttggacagctggtgctgcagcttattatgtgggttatcttcaacctaggacttttctattaaaatataatgaaaatggaaccattacagatgctgtagactgtgcacttgaccctctctcagaaacaaagtgtacgttgaaatccttcactgtagaaaaaggaatctatcaaacttctaactttagagtccaaccaacagaatctattgttagatttcctaatattacaaacttgtgcccttttggtgaagtttttaacgccaccagatttgcatctgtttatgcttggaacaggaagagaatcagcaactgtgttgctgattattctgtcctatataattccgcatcattttccacttttaagtgttatggagtgtctcctactaaattaaatgatctctgctttactaatgtctatgcagattcatttgtaattagaggtgatgaagtcagacaaatcgctccagggcaaactggaaagattgctgattataattataaattaccagatgattttacaggctgcgttatagcttggaactctaacaatcttgattctaaggttggtggtaattataattacctgtatagattgtttaggaagtctaatctcaaaccttttgagagagatatttcaactgaaatctatcaggccggtagcacaccttgtaatggtgttgaaggttttaattgttactttcctttacaatcatatggtttccaacccactaatggtgttggttaccaaccatacagagtagtagtactttcttttgaacttctacatgcaccagcaactgtttgtggacctaaaaagtctactaatttggttaaaaacaaatgtgtcaatttcaacttcaatggtttaacaggcacaggtgttcttactgagtctaacaaaaagtttctgcctttccaacaatttggcagagacattgctgacactactgatgctgtccgtgatccacagacacttgagattcttgacattacaccatgttcttttggtggtgtcagtgttataacaccaggaacaaatacttctaaccaggttgctgttctttatcaggatgttaactgcacagaagtccctgttgctattcatgcagatcaacttactcctacttggcgtgtttattctacaggttctaatgtttttcaaacacgtgcaggctgtttaataggggctgaacatgtcaacaactcatatgagtgtgacatacccattggtgcaggtatatgcgctagttatcagactcagactaattctcctcggcgggcacgtagtgtagctagtcaatccatcattgcctacactatgtcacttggtgcagaaaattcagttgcttactctaataactctattgccatacccacaaattttactattagtgttaccacagaaattctaccagtgtctatgaccaagacatcagtagattgtacaatgtacatttgtggtgattcaactgaatgcagcaatcttttgttgcaatatggcagtttttgtacacaattaaaccgtgctttaactggaatagctgttgaacaagacaaaaacacccaagaagtttttgcacaagtcaaacaaatttacaaaacaccaccaattaaagattttggtggttttaatttttcacaaatattaccagatccatcaaaaccaagcaagaggtcatttattgaagatctacttttcaacaaagtgacacttgcagatgctggcttcatcaaacaatatggtgattgccttggtgatattgctgctagagacctcatttgtgcacaaaagtttaacggccttactgttttgccacctttgctcacagatgaaatgattgctcaatacacttctgcactgttagcgggtacaatcacttctggttggacctttggtgcaggtgctgcattacaaataccatttgctatgcaaatggcttataggtttaatggtattggagttacacagaatgttctctatgagaaccaaaaattgattgccaaccaatttaatagtgctattggcaaaattcaagactcactttcttccacagcaagtgcacttggaaaacttcaagatgtggtcaaccaaaatgcacaagctttaaacacgcttgttaaacaacttagctccaattttggtgcaatttcaagtgttttaaatgatatcctttcacgtcttgacaaagttgaggctgaagtgcaaattgataggttgatcacaggcagacttcaaagtttgcagacatatgtgactcaacaattaattagagctgcagaaatcagagcttctgctaatcttgctgctactaaaatgtcagagtgtgtacttggacaatcaaaaagagttgatttttgtggaaagggctatcatcttatgtccttccctcagtcagcacctcatggtgtagtcttcttgcatgtgacttatgtccctgcacaagaaaagaacttcacaactgctcctgccatttgtcatgatggaaaagcacactttcctcgtgaaggtgtctttgtttcaaatggcacacactggtttgtaacacaaaggaatttttatgaaccacaaatcattactacagacaacacatttgtgtctggtaactgtgatgttgtaataggaattgtcaacaacacagtttatgatcctttgcaacctgaattagactcattcaaggaggagttagataaatattttaagaatcatacatcaccagatgttgatttaggtgacatctctggcattaatgcttcagttgtaaacattcaaaaagaaattgaccgcctcaatgaggttgccaagaatttaaatgaatctctcatcgatctccaagaacttggaaagtatgagcagtatataaaa

SEQ ID NO: 42 - protein, 1211 aa, SARS-CoV-2
  REGION 1..1211: note = SARS-CoV-2 spike protein ectodomain (ECD) with nativesignal peptide
MFVFLVLLPLVSSQCVNLTTRTQLPPAYTNSFTRGVYYPDKVFRSSVLHSTQDLFLPFFSNVTWFHAIHVSGTNGTKRFDNPVLPFNDGVYFASTEKSNIIRGWIFGTTLDSKTQSLLIVNNATNVVIKVCEFQFCNDPFLGVYYHKNNKSWMESEFRVYSSANNCTFEYVSQPFLMDLEGKQGNFKNLREFVFKNIDGYFKIYSKHTPINLVRDLPQGFSALEPLVDLPIGINITRFQTLLALHRSYLTPGDSSSGWTAGAAAYYVGYLQPRTFLLKYNENGTITDAVDCALDPLSETKCTLKSFTVEKGIYQTSNFRVQPTESIVRFPNITNLCPFGEVFNATRFASVYAWNRKRISNCVADYSVLYNSASFSTFKCYGVSPTKLNDLCFTNVYADSFVIRGDEVRQIAPGQTGKIADYNYKLPDDFTGCVIAWNSNNLDSKVGGNYNYLYRLFRKSNLKPFERDISTEIYQAGSTPCNGVEGFNCYFPLQSYGFQPTNGVGYQPYRVVVLSFELLHAPATVCGPKKSTNLVKNKCVNFNFNGLTGTGVLTESNKKFLPFQQFGRDIADTTDAVRDPQTLEILDITPCSFGGVSVITPGTNTSNQVAVLYQDVNCTEVPVAIHADQLTPTWRVYSTGSNVFQTRAGCLIGAEHVNNSYECDIPIGAGICASYQTQTNSPRRARSVASQSIIAYTMSLGAENSVAYSNNSIAIPTNFTISVTTEILPVSMTKTSVDCTMYICGDSTECSNLLLQYGSFCTQLNRALTGIAVEQDKNTQEVFAQVKQIYKTPPIKDFGGFNFSQILPDPSKPSKRSFIEDLLFNKVTLADAGFIKQYGDCLGDIAARDLICAQKFNGLTVLPPLLTDEMIAQYTSALLAGTITSGWTFGAGAALQIPFAMQMAYRFNGIGVTQNVLYENQKLIANQFNSAIGKIQDSLSSTASALGKLQDVVNQNAQALNTLVKQLSSNFGAISSVLNDILSRLDKVEAEVQIDRLITGRLQSLQTYVTQQLIRAAEIRASANLAATKMSECVLGQSKRVDFCGKGYHLMSFPQSAPHGVVFLHVTYVPAQEKNFTTAPAICHDGKAHFPREGVFVSNGTHWFVTQRNFYEPQIITTDNTFVSGNCDVVIGIVNNTVYDPLQPELDSFKEELDKYFKNHTSPDVDLGDISGINASVVNIQKEIDRLNEVAKNLNESLIDLQELGKYEQYIK

SEQ ID NO: 43 - DNA, 3633 bp, SARS-CoV-2; identical to SEQ ID NO: 41
  misc_feature 1..3633: note = SARS-CoV-2 spike protein ectodomain (ECD) with native signalpeptide coding sequence
  source 1..3633: mol_type = other DNA

SEQ ID NO: 44 - protein, 685 aa, SARS-CoV-2
  REGION 1..685: note = SARS-CoV-2 spike protein S1 subunit with native signal peptide
MFVFLVLLPLVSSQCVNLTTRTQLPPAYTNSFTRGVYYPDKVFRSSVLHSTQDLFLPFFSNVTWFHAIHVSGTNGTKRFDNPVLPFNDGVYFASTEKSNIIRGWIFGTTLDSKTQSLLIVNNATNVVIKVCEFQFCNDPFLGVYYHKNNKSWMESEFRVYSSANNCTFEYVSQPFLMDLEGKQGNFKNLREFVFKNIDGYFKIYSKHTPINLVRDLPQGFSALEPLVDLPIGINITRFQTLLALHRSYLTPGDSSSGWTAGAAAYYVGYLQPRTFLLKYNENGTITDAVDCALDPLSETKCTLKSFTVEKGIYQTSNFRVQPTESIVRFPNITNLCPFGEVFNATRFASVYAWNRKRISNCVADYSVLYNSASFSTFKCYGVSPTKLNDLCFTNVYADSFVIRGDEVRQIAPGQTGKIADYNYKLPDDFTGCVIAWNSNNLDSKVGGNYNYLYRLFRKSNLKPFERDISTEIYQAGSTPCNGVEGFNCYFPLQSYGFQPTNGVGYQPYRVVVLSFELLHAPATVCGPKKSTNLVKNKCVNFNFNGLTGTGVLTESNKKFLPFQQFGRDIADTTDAVRDPQTLEILDITPCSFGGVSVITPGTNTSNQVAVLYQDVNCTEVPVAIHADQLTPTWRVYSTGSNVFQTRAGCLIGAEHVNNSYECDIPIGAGICASYQTQTNSPRRAR

SEQ ID NO: 45 - DNA, 2055 bp, SARS-CoV-2
  misc_feature 1..2055: note = SARS-CoV-2 spike protein S1 subunit with native signalpeptide coding sequence
  source 1..2055: mol_type = other DNA
atgtttgtttttcttgttttattgccattagtctctagtcagtgtgttaatcttacaaccagaactcaattaccccctgcatacactaattctttcacacgtggtgtttattaccctgacaaagttttcagatcctcagttttacattcaactcaggacttgttcttacctttcttttccaatgttacttggttccatgctatacatgtctctgggaccaatggtactaagaggtttgataaccctgtcctaccatttaatgatggtgtttattttgcttccactgagaagtctaacataataagaggctggatttttggtactactttagattcgaagacccagtccctacttattgttaataacgctactaatgttgttattaaagtctgtgaatttcaattttgtaatgatccatttttgggtgtttattaccacaaaaacaacaaaagttggatggaaagtgagttcagagtttattctagtgcgaataattgcacttttgaatatgtctctcagccttttcttatggaccttgaaggaaaacagggtaatttcaaaaatcttagggaatttgtgtttaagaatattgatggttattttaaaatatattctaagcacacgcctattaatttagtgcgtgatctccctcagggtttttcggctttagaaccattggtagatttgccaataggtattaacatcactaggtttcaaactttacttgctttacatagaagttatttgactcctggtgattcttcttcaggttggacagctggtgctgcagcttattatgtgggttatcttcaacctaggacttttctattaaaatataatgaaaatggaaccattacagatgctgtagactgtgcacttgaccctctctcagaaacaaagtgtacgttgaaatccttcactgtagaaaaaggaatctatcaaacttctaactttagagtccaaccaacagaatctattgttagatttcctaatattacaaacttgtgcccttttggtgaagtttttaacgccaccagatttgcatctgtttatgcttggaacaggaagagaatcagcaactgtgttgctgattattctgtcctatataattccgcatcattttccacttttaagtgttatggagtgtctcctactaaattaaatgatctctgctttactaatgtctatgcagattcatttgtaattagaggtgatgaagtcagacaaatcgctccagggcaaactggaaagattgctgattataattataaattaccagatgattttacaggctgcgttatagcttggaattctaacaatcttgattctaaggttggtggtaattataattacctgtatagattgtttaggaagtctaatctcaaaccttttgagagagatatttcaactgaaatctatcaggccggtagcacaccttgtaatggtgttgaaggttttaattgttactttcctttacaatcatatggtttccaacccactaatggtgttggttaccaaccatacagagtagtagtactttcttttgaacttctacatgcaccagcaactgtttgtggacctaaaaagtctactaatttggttaaaaacaaatgtgtcaatttcaacttcaatggtttaacaggcacaggtgttcttactgagtctaacaaaaagtttctgcctttccaacaatttggcagagacattgctgacactactgatgctgtccgtgatccacagacacttgagattcttgacattacaccatgttcttttggtggtgtcagtgttataacaccaggaacaaatacttctaaccaggttgctgttctttatcaggatgttaactgcacagaagtccctgttgctattcatgcagatcaacttactcctacttggcgtgtttattctacaggttctaatgtttttcaaacacgtgcaggctgtttaataggggctgaacatgtcaacaactcatatgagtgtgacatacccattggtgcaggtatatgcgctagttatcagactcagactaattctcctcggcgggcacgt

SEQ ID NO: 46 - DNA, 39 bp, synthetic construct
  misc_feature 1..39: note = Exemplary 5-Prime-UTR DNA Sequence
  source 1..39: mol_type = other DNA
gaaataagagagaaaagaagagtaagaagaaatataaga

SEQ ID NO: 47 - RNA, 39 nt, synthetic construct
  misc_feature 1..39: note = Exemplary 5-Prime-UTR RNA Sequence
  source 1..39: mol_type = other RNA
gaaataagagagaaaagaagagtaagaagaaatataaga

SEQ ID NO: 48 - DNA, 44 bp, synthetic construct
  misc_feature 1..44: note = Exemplary 5-Prime-UTR DNA Sequence
  source 1..44: mol_type = other DNA
cttgttctttttgcagaagctcagaataaacgctcaactttggc

SEQ ID NO: 49 - RNA, 44 nt, synthetic construct
  misc_feature 1..44: note = Exemplary 5-Prime-UTR RNA Sequence
  source 1..44: mol_type = other RNA
cttgttctttttgcagaagctcagaataaacgctcaactttggc

SEQ ID NO: 50 - DNA, 100 bp, synthetic construct
  misc_feature 1..100: note = Exemplary 5-Prime-UTR DNA Sequence
  source 1..100: mol_type = other DNA
gcaggagccagggctgggcataaaagtcagggcagagccatctattgcttacatttgcttctgacacaactgtgttcactagcaacctcaaacagacacc

SEQ ID NO: 51 - RNA, 100 nt, synthetic construct
  misc_feature 1..100: note = Exemplary 5-Prime-UTR RNA Sequence
  source 1..100: mol_type = other RNA
gcaggagccagggctgggcataaaagtcagggcagagccatctattgcttacatttgcttctgacacaactgtgttcactagcaacctcaaacagacacc

SEQ ID NO: 52 - DNA, 110 bp, synthetic construct
  misc_feature 1..110: note = Exemplary 3-Prime-UTR DNA Sequence
  source 1..110: mol_type = other DNA
gctggagcctcggtggccatgcttcttgccccttgggcctccccccagcccctcctccccttcctgcacccgtacccccgtggtctttgaataaagtctgagtgggcggc

SEQ ID NO: 53 - RNA, 110 nt, synthetic construct
  misc_feature 1..110: note = Exemplary 3-Prime-UTR RNA Sequence
  source 1..110: mol_type = other RNA
gctggagcctcggtggccatgcttcttgccccttgggcctccccccagcccctcctccccttcctgcacccgtacccccgtggtctttgaataaagtctgagtgggcggc

SEQ ID NO: 54 - DNA, 132 bp, synthetic construct
  misc_feature 1..132: note = Exemplary 3-Prime-UTR DNA Sequence
  source 1..132: mol_type = other DNA
gctcgctttcttgctgtccaatttctattaaaggttcctttgttccctaagtccaactactaaactgggggatattatgaagggccttgagcatctggattctgcctaataaaaaacatttattttcattgc

SEQ ID NO: 55 - RNA, 132 nt, synthetic construct
  misc_feature 1..132: note = Exemplary 3-Prime-UTR RNA Sequence
  source 1..132: mol_type = other RNA
gctcgctttcttgctgtccaatttctattaaaggttcctttgttccctaagtccaactactaaactgggggatattatgaagggccttgagcatctggattctgcctaataaaaaacatttattttcattgc

SEQ ID NO: 56 - DNA, 278 bp, synthetic construct
  misc_feature 1..278: note = Exemplary 3-Prime-UTR DNA Sequence
  source 1..278: mol_type = other DNA
ctggtactgcatgcacgcaatgctagctgcccctttcccgtcctgggtaccccgagtctcccccgacctcgggtcccaggtatgctcccacctccacctgccccactcaccacctctgctagttccagacacctcccaagcacgcagcaatgcagctcaaaacgcttagcctagccacacccccacgggaaacagcagtgattaacctttagcaataaacgaaagtttaactaagctatactaaccccagggttggtcaatttcgtgccagccacacc

SEQ ID NO: 57 - RNA, 278 nt, synthetic construct
  misc_feature 1..278: note = Exemplary 3-Prime-UTR RNA Sequence
  source 1..278: mol_type = other RNA
ctggtactgcatgcacgcaatgctagctgcccctttcccgtcctgggtaccccgagtctcccccgacctcgggtcccaggtatgctcccacctccacctgccccactcaccacctctgctagttccagacacctcccaagcacgcagcaatgcagctcaaaacgcttagcctagccacacccccacgggaaacagcagtgattaacctttagcaataaacgaaagtttaactaagctatactaaccccagggttggtcaatttcgtgccagccacacc

SEQ ID NO: 58 - DNA, 24 bp, synthetic construct
  misc_feature 1..24: note = stem-loop sequence
  source 1..24: mol_type = other DNA
caaaggctcttttcagagccacca

SEQ ID NO: 59 - RNA, 24 nt, synthetic construct
  misc_feature 1..24: note = stem-loop sequence
  source 1..24: mol_type = other RNA
caaaggctcttttcagagccacca

SEQ ID NO: 60 - DNA, 1075 bp, synthetic construct
  misc_feature 1..1075: note = mRNA-001 DNA
  source 1..1075: mol_type = other DNA
ggggggatccaagcttagcttgttctttttgcagaagctcagaataaacgctcaactttggcgccgccaccatggactggacctggattctcttcttggtggcagcagccacgcgagtccactccagagtccaaccaacagaatctattgttagatttcctaatattacaaacttgtgcccttttggtgaagtttttaacgccaccagatttgcatctgtttatgcttggaacaggaagagaatcagcaactgtgttgctgattattctgtcctatataattccgcatcattttccacttttaagtgttatggagtgtctcctactaaattaaatgatctctgctttactaatgtctatgcagattcatttgtaattagaggtgatgaagtcagacaaatcgctccagggcaaactggaaagattgctgattataattataaattaccagatgattttacaggctgcgttatagcttggaactctaacaatcttgattctaaggttggtggtaattataattacctgtatagattgtttaggaagtctaatctcaaaccttttgagagagatatttcaactgaaatctatcaggccggtagcacaccttgtaatggtgttgaaggttttaattgttactttcctttacaatcatatggtttccaacccactaatggtgttggttaccaaccatacagagtagtagtactttcttttgaacttctacatgcaccagcaactgtttgtggacctaaaaagtctactaatttggttaaaaacaaatgtgtcaatttctgataagaattctaggctggagcctcggtggccatgcttcttgccccttgggcctccccccagcccctcctccccttcctgcacccgtacccccgtggtctttgaataaagtctgagtgggcggcactagtaaaaaaaaaaaaaaaaaaaaaaaaaaaaaaaaaaaaaaaaaaaaaaaaaaaaaaaaaaaaaaaaaaaaaaaaaaaaaaaaaaaaaaaaaaaaaaaaaaaaaaaaaaaaaaaaaaaaaaaaaaaaaaaaaaaaaaaaaaaaaaaaaaaaaa

SEQ ID NO: 61 - RNA, 1076 nt, synthetic construct
  misc_feature 1..1076: note = mRNA-001
  source 1..1076: mol_type = other RNA
gggggggatccaagcttagcttgttctttttgcagaagctcagaataaacgctcaactttggcgccgccaccatggactggacctggattctcttcttggtggcagcagccacgcgagtccactccagagtccaaccaacagaatctattgttagatttcctaatattacaaacttgtgcccttttggtgaagtttttaacgccaccagatttgcatctgtttatgcttggaacaggaagagaatcagcaactgtgttgctgattattctgtcctatataattccgcatcattttccacttttaagtgttatggagtgtctcctactaaattaaatgatctctgctttactaatgtctatgcagattcatttgtaattagaggtgatgaagtcagacaaatcgctccagggcaaactggaaagattgctgattataattataaattaccagatgattttacaggctgcgttatagcttggaactctaacaatcttgattctaaggttggtggtaattataattacctgtatagattgtttaggaagtctaatctcaaaccttttgagagagatatttcaactgaaatctatcaggccggtagcacaccttgtaatggtgttgaaggttttaattgttactttcctttacaatcatatggtttccaacccactaatggtgttggttaccaaccatacagagtagtagtactttcttttgaacttctacatgcaccagcaactgtttgtggacctaaaaagtctactaatttggttaaaaacaaatgtgtcaatttctgataagaattctaggctggagcctcggtggccatgcttcttgccccttgggcctccccccagcccctcctccccttcctgcacccgtacccccgtggtctttgaataaagtctgagtgggcggcactagtaaaaaaaaaaaaaaaaaaaaaaaaaaaaaaaaaaaaaaaaaaaaaaaaaaaaaaaaaaaaaaaaaaaaaaaaaaaaaaaaaaaaaaaaaaaaaaaaaaaaaaaaaaaaaaaaaaaaaaaaaaaaaaaaaaaaaaaaaaaaaaaaaaaaaa

SEQ ID NO: 62 - DNA, 1003 bp, synthetic construct
  misc_feature 1..1003: note = mRNA-002 DNA
  source 1..1003: mol_type = other DNA
ggggggatccaagcttagcttgttctttttgcagaagctcagaataaacgctcaactttggcgccgccaccatggactggacctggattctcttcttggtggcagcagccacgcgagtccactccaatattacaaacttgtgcccttttggtgaagtttttaacgccaccagatttgcatctgtttatgcttggaacaggaagagaatcagcaactgtgttgctgattattctgtcctatataattccgcatcattttccacttttaagtgttatggagtgtctcctactaaattaaatgatctctgctttactaatgtctatgcagattcatttgtaattagaggtgatgaagtcagacaaatcgctccagggcaaactggaaagattgctgattataattataaattaccagatgattttacaggctgcgttatagcttggaactctaacaatcttgattctaaggttggtggtaattataattacctgtatagattgtttaggaagtctaatctcaaaccttttgagagagatatttcaactgaaatctatcaggccggtagcacaccttgtaatggtgttgaaggttttaattgttactttcctttacaatcatatggtttccaacccactaatggtgttggttaccaaccatacagagtagtagtactttcttttgaacttctacatgcaccagcaactgtttgtggacctaaaaagtgataagaattctaggctggagcctcggtggccatgcttcttgccccttgggcctccccccagcccctcctccccttcctgcacccgtacccccgtggtctttgaataaagtctgagtgggcggcactagtaaaaaaaaaaaaaaaaaaaaaaaaaaaaaaaaaaaaaaaaaaaaaaaaaaaaaaaaaaaaaaaaaaaaaaaaaaaaaaaaaaaaaaaaaaaaaaaaaaaaaaaaaaaaaaaaaaaaaaaaaaaaaaaaaaaaaaaaaaaaaaaaaaaaaa

SEQ ID NO: 63 - RNA, 1004 nt, synthetic construct
  misc_feature 1..1004: note = mRNA-002
  source 1..1004: mol_type = other RNA
gggggggatccaagcttagcttgttctttttgcagaagctcagaataaacgctcaactttggcgccgccaccatggactggacctggattctcttcttggtggcagcagccacgcgagtccactccaatattacaaacttgtgcccttttggtgaagtttttaacgccaccagatttgcatctgtttatgcttggaacaggaagagaatcagcaactgtgttgctgattattctgtcctatataattccgcatcattttccacttttaagtgttatggagtgtctcctactaaattaaatgatctctgctttactaatgtctatgcagattcatttgtaattagaggtgatgaagtcagacaaatcgctccagggcaaactggaaagattgctgattataattataaattaccagatgattttacaggctgcgttatagcttggaactctaacaatcttgattctaaggttggtggtaattataattacctgtatagattgtttaggaagtctaatctcaaaccttttgagagagatatttcaactgaaatctatcaggccggtagcacaccttgtaatggtgttgaaggttttaattgttactttcctttacaatcatatggtttccaacccactaatggtgttggttaccaaccatacagagtagtagtactttcttttgaacttctacatgcaccagcaactgtttgtggacctaaaaagtgataagaattctaggctggagcctcggtggccatgcttcttgccccttgggcctccccccagcccctcctccccttcctgcacccgtacccccgtggtctttgaataaagtctgagtgggcggcactagtaaaaaaaaaaaaaaaaaaaaaaaaaaaaaaaaaaaaaaaaaaaaaaaaaaaaaaaaaaaaaaaaaaaaaaaaaaaaaaaaaaaaaaaaaaaaaaaaaaaaaaaaaaaaaaaaaaaaaaaaaaaaaaaaaaaaaaaaaaaaaaaaaaaaaa

SEQ ID NO: 64 - DNA, 988 bp, synthetic construct
  misc_feature 1..988: note = mRNA-003 DNA
  source 1..988: mol_type = other DNA
ggggggatccaagcttagcttgttctttttgcagaagctcagaataaacgctcaactttggcgccgccaccatggactggacctggattctcttcttggtggcagcagccacgcgagtccactccaatattacaaacttgtgcccttttggtgaagtttttaacgccaccagatttgcatctgtttatgcttggaacaggaagagaatcagcaactgtgttgctgattattctgtcctatataattccgcatcattttccacttttaagtgttatggagtgtctcctactaaattaaatgatctctgctttactaatgtctatgcagattcatttgtaattagaggtgatgaagtcagacaaatcgctccagggcaaactggaaagattgctgattataattataaattaccagatgattttacaggctgcgttatagcttggaactctaacaatcttgattctaaggttggtggtaattataattacctgtatagattgtttaggaagtctaatctcaaaccttttgagagagatatttcaactgaaatctatcaggccggtagcacaccttgtaatggtgttgaaggttttaattgttactttcctttacaatcatatggtttccaacccactaatggtgttggttaccaaccatacagagtagtagtactttcttttgaacttctacatgcaccagcaactgtttgataagaattctaggctggagcctcggtggccatgcttcttgccccttgggcctccccccagcccctcctccccttcctgcacccgtacccccgtggtctttgaataaagtctgagtgggcggcactagtaaaaaaaaaaaaaaaaaaaaaaaaaaaaaaaaaaaaaaaaaaaaaaaaaaaaaaaaaaaaaaaaaaaaaaaaaaaaaaaaaaaaaaaaaaaaaaaaaaaaaaaaaaaaaaaaaaaaaaaaaaaaaaaaaaaaaaaaaaaaaaaaaaaaaa

SEQ ID NO: 65 - RNA, 989 nt, synthetic construct
  misc_feature 1..989: note = mRNA-003
  source 1..989: mol_type = other RNA
gggggggatccaagcttagcttgttctttttgcagaagctcagaataaacgctcaactttggcgccgccaccatggactggacctggattctcttcttggtggcagcagccacgcgagtccactccaatattacaaacttgtgcccttttggtgaagtttttaacgccaccagatttgcatctgtttatgcttggaacaggaagagaatcagcaactgtgttgctgattattctgtcctatataattccgcatcattttccacttttaagtgttatggagtgtctcctactaaattaaatgatctctgctttactaatgtctatgcagattcatttgtaattagaggtgatgaagtcagacaaatcgctccagggcaaactggaaagattgctgattataattataaattaccagatgattttacaggctgcgttatagcttggaactctaacaatcttgattctaaggttggtggtaattataattacctgtatagattgtttaggaagtctaatctcaaaccttttgagagagatatttcaactgaaatctatcaggccggtagcacaccttgtaatggtgttgaaggttttaattgttactttcctttacaatcatatggtttccaacccactaatggtgttggttaccaaccatacagagtagtagtactttcttttgaacttctacatgcaccagcaactgtttgataagaattctaggctggagcctcggtggccatgcttcttgccccttgggcctccccccagcccctcctccccttcctgcacccgtacccccgtggtctttgaataaagtctgagtgggcggcactagtaaaaaaaaaaaaaaaaaaaaaaaaaaaaaaaaaaaaaaaaaaaaaaaaaaaaaaaaaaaaaaaaaaaaaaaaaaaaaaaaaaaaaaaaaaaaaaaaaaaaaaaaaaaaaaaaaaaaaaaaaaaaaaaaaaaaaaaaaaaaaaaaaaaaaa

SEQ ID NO: 66 - DNA, 1039 bp, synthetic construct
  misc_feature 1..1039: note = mRNA-004 DNA
  source 1..1039: mol_type = other DNA
ggggggatccaagcttagcttgttctttttgcagaagctcagaataaacgctcaactttggcgccgccaccatggactggacctggattctcttcttggtggcagcagccacgcgagtccactccagagtccaaccaacagaatctattgttagatttcctaatattacaaacttgtgcccttttggtgaagtttttaacgccaccagatttgcatctgtttatgcttggaacaggaagagaatcagcaactgtgttgctgattattctgtcctatataattccgcatcattttccacttttaagtgttatggagtgtctcctactaaattaaatgatctctgctttactaatgtctatgcagattcatttgtaattagaggtgatgaagtcagacaaatcgctccagggcaaactggaaagattgctgattataattataaattaccagatgattttacaggctgcgttatagcttggaactctaacaatcttgattctaaggttggtggtaattataattacctgtatagattgtttaggaagtctaatctcaaaccttttgagagagatatttcaactgaaatctatcaggccggtagcacaccttgtaatggtgttgaaggttttaattgttactttcctttacaatcatatggtttccaacccactaatggtgttggttaccaaccatacagagtagtagtactttcttttgaacttctacatgcaccagcaactgtttgtggacctaaaaagtgataagaattctaggctggagcctcggtggccatgcttcttgccccttgggcctccccccagcccctcctccccttcctgcacccgtacccccgtggtctttgaataaagtctgagtgggcggcactagtaaaaaaaaaaaaaaaaaaaaaaaaaaaaaaaaaaaaaaaaaaaaaaaaaaaaaaaaaaaaaaaaaaaaaaaaaaaaaaaaaaaaaaaaaaaaaaaaaaaaaaaaaaaaaaaaaaaaaaaaaaaaaaaaaaaaaaaaaaaaaaaaaaaaaa

SEQ ID NO: 67 - RNA, 1040 nt, synthetic construct
  misc_feature 1..1040: note = mRNA-004
  source 1..1040: mol_type = other RNA
gggggggatccaagcttagcttgttctttttgcagaagctcagaataaacgctcaactttggcgccgccaccatggactggacctggattctcttcttggtggcagcagccacgcgagtccactccagagtccaaccaacagaatctattgttagatttcctaatattacaaacttgtgcccttttggtgaagtttttaacgccaccagatttgcatctgtttatgcttggaacaggaagagaatcagcaactgtgttgctgattattctgtcctatataattccgcatcattttccacttttaagtgttatggagtgtctcctactaaattaaatgatctctgctttactaatgtctatgcagattcatttgtaattagaggtgatgaagtcagacaaatcgctccagggcaaactggaaagattgctgattataattataaattaccagatgattttacaggctgcgttatagcttggaactctaacaatcttgattctaaggttggtggtaattataattacctgtatagattgtttaggaagtctaatctcaaaccttttgagagagatatttcaactgaaatctatcaggccggtagcacaccttgtaatggtgttgaaggttttaattgttactttcctttacaatcatatggtttccaacccactaatggtgttggttaccaaccatacagagtagtagtactttcttttgaacttctacatgcaccagcaactgtttgtggacctaaaaagtgataagaattctaggctggagcctcggtggccatgcttcttgccccttgggcctccccccagcccctcctccccttcctgcacccgtacccccgtggtctttgaataaagtctgagtgggcggcactagtaaaaaaaaaaaaaaaaaaaaaaaaaaaaaaaaaaaaaaaaaaaaaaaaaaaaaaaaaaaaaaaaaaaaaaaaaaaaaaaaaaaaaaaaaaaaaaaaaaaaaaaaaaaaaaaaaaaaaaaaaaaaaaaaaaaaaaaaaaaaaaaaaaaaaa

SEQ ID NO: 68 - DNA, 1075 bp, synthetic construct
  misc_feature 1..1075: note = mRNA-005 DNA
  source 1..1075: mol_type = other DNA
ggggggatccaagcttagcttgttctttttgcagaagctcagaataaacgctcaactttggcgccgccaccatggactggacctggattctcttcttggtggcagcagccacgcgagtccactccagagtccaaccaacagaatctattgttagatttcctaatattacaaacttgtgcccttttggtgaagtttttaacgccaccagatttgcatctgtttatgcttggaacaggaagagaatcagcaactgtgttgctgattattctgtcctatataattccgcatcattttccacttttaagtgttatggagtgtctcctactaaattaaatgatctctgctttactaatgtctatgcagattcatttgtaattagaggtgatgaagtcagacaaatcgctccagggcaaactggaaagattgctgattataattataaattaccagatgattttacaggctgcgttatagcttggaactctaacaatcttgattctaaggttggtggtaattataattacctgtatagattgtttaggaagtctaatctcaaaccttttgagagagatatttcaactgaaatctatcaggccggtagcacaccttgtaatggtgttgaaggttttaattgttactttcctttacaatcatatggtttccaacccactactggtgttggttaccaaccatacagagtagtagtactttcttttgaacttctacatgcaccagcaactgtttgtggacctaaaaagtctactaatttggttaaaaacaaatgtgtcaatttctgataagaattctaggctggagcctcggtggccatgcttcttgccccttgggcctccccccagcccctcctccccttcctgcacccgtacccccgtggtctttgaataaagtctgagtgggcggcactagtaaaaaaaaaaaaaaaaaaaaaaaaaaaaaaaaaaaaaaaaaaaaaaaaaaaaaaaaaaaaaaaaaaaaaaaaaaaaaaaaaaaaaaaaaaaaaaaaaaaaaaaaaaaaaaaaaaaaaaaaaaaaaaaaaaaaaaaaaaaaaaaaaaaaaa

SEQ ID NO: 69 - RNA, 1076 nt, synthetic construct
  misc_feature 1..1076: note = mRNA-005
  source 1..1076: mol_type = other RNA
gggggggatccaagcttagcttgttctttttgcagaagctcagaataaacgctcaactttggcgccgccaccatggactggacctggattctcttcttggtggcagcagccacgcgagtccactccagagtccaaccaacagaatctattgttagatttcctaatattacaaacttgtgcccttttggtgaagtttttaacgccaccagatttgcatctgtttatgcttggaacaggaagagaatcagcaactgtgttgctgattattctgtcctatataattccgcatcattttccacttttaagtgttatggagtgtctcctactaaattaaatgatctctgctttactaatgtctatgcagattcatttgtaattagaggtgatgaagtcagacaaatcgctccagggcaaactggaaagattgctgattataattataaattaccagatgattttacaggctgcgttatagcttggaactctaacaatcttgattctaaggttggtggtaattataattacctgtatagattgtttaggaagtctaatctcaaaccttttgagagagatatttcaactgaaatctatcaggccggtagcacaccttgtaatggtgttgaaggttttaattgttactttcctttacaatcatatggtttccaacccactactggtgttggttaccaaccatacagagtagtagtactttcttttgaacttctacatgcaccagcaactgtttgtggacctaaaaagtctactaatttggttaaaaacaaatgtgtcaatttctgataagaattctaggctggagcctcggtggccatgcttcttgccccttgggcctccccccagcccctcctccccttcctgcacccgtacccccgtggtctttgaataaagtctgagtgggcggcactagtaaaaaaaaaaaaaaaaaaaaaaaaaaaaaaaaaaaaaaaaaaaaaaaaaaaaaaaaaaaaaaaaaaaaaaaaaaaaaaaaaaaaaaaaaaaaaaaaaaaaaaaaaaaaaaaaaaaaaaaaaaaaaaaaaaaaaaaaaaaaaaaaaaaaaa

SEQ ID NO: 70 - DNA, 1060 bp, synthetic construct
  misc_feature 1..1060: note = mRNA-006 DNA
  source 1..1060: mol_type = other DNA
ggggggatccaagcttagcttgttctttttgcagaagctcagaataaacgctcaactttggcgccgccaccatgtttgtttttcttgttttattgccattagtctctagtagagtccaaccaacagaatctattgttagatttcctaatattacaaacttgtgcccttttggtgaagtttttaacgccaccagatttgcatctgtttatgcttggaacaggaagagaatcagcaactgtgttgctgattattctgtcctatataattccgcatcattttccacttttaagtgttatggagtgtctcctactaaattaaatgatctctgctttactaatgtctatgcagattcatttgtaattagaggtgatgaagtcagacaaatcgctccagggcaaactggaaagattgctgattataattataaattaccagatgattttacaggctgcgttatagcttggaactctaacaatcttgattctaaggttggtggtaattataattacctgtatagattgtttaggaagtctaatctcaaaccttttgagagagatatttcaactgaaatctatcaggccggtagcacaccttgtaatggtgttgaaggttttaattgttactttcctttacaatcatatggtttccaacccactaatggtgttggttaccaaccatacagagtagtagtactttcttttgaacttctacatgcaccagcaactgtttgtggacctaaaaagtctactaatttggttaaaaacaaatgtgtcaatttctgataagaattctaggctggagcctcggtggccatgcttcttgccccttgggcctccccccagcccctcctccccttcctgcacccgtacccccgtggtctttgaataaagtctgagtgggcggcactagtaaaaaaaaaaaaaaaaaaaaaaaaaaaaaaaaaaaaaaaaaaaaaaaaaaaaaaaaaaaaaaaaaaaaaaaaaaaaaaaaaaaaaaaaaaaaaaaaaaaaaaaaaaaaaaaaaaaaaaaaaaaaaaaaaaaaaaaaaaaaaaaaaaaaaa

SEQ ID NO: 71 - RNA, 1061 nt, synthetic construct
  misc_feature 1..1061: note = mRNA-006
  source 1..1061: mol_type = other RNA
gggggggatccaagcttagcttgttctttttgcagaagctcagaataaacgctcaactttggcgccgccaccatgtttgtttttcttgttttattgccattagtctctagtagagtccaaccaacagaatctattgttagatttcctaatattacaaacttgtgcccttttggtgaagtttttaacgccaccagatttgcatctgtttatgcttggaacaggaagagaatcagcaactgtgttgctgattattctgtcctatataattccgcatcattttccacttttaagtgttatggagtgtctcctactaaattaaatgatctctgctttactaatgtctatgcagattcatttgtaattagaggtgatgaagtcagacaaatcgctccagggcaaactggaaagattgctgattataattataaattaccagatgattttacaggctgcgttatagcttggaactctaacaatcttgattctaaggttggtggtaattataattacctgtatagattgtttaggaagtctaatctcaaaccttttgagagagatatttcaactgaaatctatcaggccggtagcacaccttgtaatggtgttgaaggttttaattgttactttcctttacaatcatatggtttccaacccactaatggtgttggttaccaaccatacagagtagtagtactttcttttgaacttctacatgcaccagcaactgtttgtggacctaaaaagtctactaatttggttaaaaacaaatgtgtcaatttctgataagaattctaggctggagcctcggtggccatgcttcttgccccttgggcctccccccagcccctcctccccttcctgcacccgtacccccgtggtctttgaataaagtctgagtgggcggcactagtaaaaaaaaaaaaaaaaaaaaaaaaaaaaaaaaaaaaaaaaaaaaaaaaaaaaaaaaaaaaaaaaaaaaaaaaaaaaaaaaaaaaaaaaaaaaaaaaaaaaaaaaaaaaaaaaaaaaaaaaaaaaaaaaaaaaaaaaaaaaaaaaaaaaaa

SEQ ID NO: 72 - DNA, 988 bp, synthetic construct
  misc_feature 1..988: note = mRNA-007 DNA
  source 1..988: mol_type = other DNA
ggggggatccaagcttagcttgttctttttgcagaagctcagaataaacgctcaactttggcgccgccaccatgtttgtttttcttgttttattgccattagtctctagtaatattacaaacttgtgcccttttggtgaagtttttaacgccaccagatttgcatctgtttatgcttggaacaggaagagaatcagcaactgtgttgctgattattctgtcctatataattccgcatcattttccacttttaagtgttatggagtgtctcctactaaattaaatgatctctgctttactaatgtctatgcagattcatttgtaattagaggtgatgaagtcagacaaatcgctccagggcaaactggaaagattgctgattataattataaattaccagatgattttacaggctgcgttatagcttggaactctaacaatcttgattctaaggttggtggtaattataattacctgtatagattgtttaggaagtctaatctcaaaccttttgagagagatatttcaactgaaatctatcaggccggtagcacaccttgtaatggtgttgaaggttttaattgttactttcctttacaatcatatggtttccaacccactaatggtgttggttaccaaccatacagagtagtagtactttcttttgaacttctacatgcaccagcaactgtttgtggacctaaaaagtgataagaattctaggctggagcctcggtggccatgcttcttgccccttgggcctccccccagcccctcctccccttcctgcacccgtacccccgtggtctttgaataaagtctgagtgggcggcactagtaaaaaaaaaaaaaaaaaaaaaaaaaaaaaaaaaaaaaaaaaaaaaaaaaaaaaaaaaaaaaaaaaaaaaaaaaaaaaaaaaaaaaaaaaaaaaaaaaaaaaaaaaaaaaaaaaaaaaaaaaaaaaaaaaaaaaaaaaaaaaaaaaaaaaa

SEQ ID NO: 73 - RNA, 989 nt, synthetic construct
  misc_feature 1..989: note = mRNA-007
  source 1..989: mol_type = other RNA
gggggggatccaagcttagcttgttctttttgcagaagctcagaataaacgctcaactttggcgccgccaccatgtttgtttttcttgttttattgccattagtctctagtaatattacaaacttgtgcccttttggtgaagtttttaacgccaccagatttgcatctgtttatgcttggaacaggaagagaatcagcaactgtgttgctgattattctgtcctatataattccgcatcattttccacttttaagtgttatggagtgtctcctactaaattaaatgatctctgctttactaatgtctatgcagattcatttgtaattagaggtgatgaagtcagacaaatcgctccagggcaaactggaaagattgctgattataattataaattaccagatgattttacaggctgcgttatagcttggaactctaacaatcttgattctaaggttggtggtaattataattacctgtatagattgtttaggaagtctaatctcaaaccttttgagagagatatttcaactgaaatctatcaggccggtagcacaccttgtaatggtgttgaaggttttaattgttactttcctttacaatcatatggtttccaacccactaatggtgttggttaccaaccatacagagtagtagtactttcttttgaacttctacatgcaccagcaactgtttgtggacctaaaaagtgataagaattctaggctggagcctcggtggccatgcttcttgccccttgggcctccccccagcccctcctccccttcctgcacccgtacccccgtggtctttgaataaagtctgagtgggcggcactagtaaaaaaaaaaaaaaaaaaaaaaaaaaaaaaaaaaaaaaaaaaaaaaaaaaaaaaaaaaaaaaaaaaaaaaaaaaaaaaaaaaaaaaaaaaaaaaaaaaaaaaaaaaaaaaaaaaaaaaaaaaaaaaaaaaaaaaaaaaaaaaaaaaaaaa

SEQ ID NO: 74 - DNA, 973 bp, synthetic construct
  misc_feature 1..973: note = mRNA-008 DNA
  source 1..973: mol_type = other DNA
ggggggatccaagcttagcttgttctttttgcagaagctcagaataaacgctcaactttggcgccgccaccatgtttgtttttcttgttttattgccattagtctctagtaatattacaaacttgtgcccttttggtgaagtttttaacgccaccagatttgcatctgtttatgcttggaacaggaagagaatcagcaactgtgttgctgattattctgtcctatataattccgcatcattttccacttttaagtgttatggagtgtctcctactaaattaaatgatctctgctttactaatgtctatgcagattcatttgtaattagaggtgatgaagtcagacaaatcgctccagggcaaactggaaagattgctgattataattataaattaccagatgattttacaggctgcgttatagcttggaactctaacaatcttgattctaaggttggtggtaattataattacctgtatagattgtttaggaagtctaatctcaaaccttttgagagagatatttcaactgaaatctatcaggccggtagcacaccttgtaatggtgttgaaggttttaattgttactttcctttacaatcatatggtttccaacccactaatggtgttggttaccaaccatacagagtagtagtactttcttttgaacttctacatgcaccagcaactgtttgataagaattctaggctggagcctcggtggccatgcttcttgccccttgggcctccccccagcccctcctccccttcctgcacccgtacccccgtggtctttgaataaagtctgagtgggcggcactagtaaaaaaaaaaaaaaaaaaaaaaaaaaaaaaaaaaaaaaaaaaaaaaaaaaaaaaaaaaaaaaaaaaaaaaaaaaaaaaaaaaaaaaaaaaaaaaaaaaaaaaaaaaaaaaaaaaaaaaaaaaaaaaaaaaaaaaaaaaaaaaaaaaaaaa

SEQ ID NO: 75 - RNA, 974 nt, synthetic construct
  misc_feature 1..974: note = mRNA-008
  source 1..974: mol_type = other RNA
gggggggatccaagcttagcttgttctttttgcagaagctcagaataaacgctcaactttggcgccgccaccatgtttgtttttcttgttttattgccattagtctctagtaatattacaaacttgtgcccttttggtgaagtttttaacgccaccagatttgcatctgtttatgcttggaacaggaagagaatcagcaactgtgttgctgattattctgtcctatataattccgcatcattttccacttttaagtgttatggagtgtctcctactaaattaaatgatctctgctttactaatgtctatgcagattcatttgtaattagaggtgatgaagtcagacaaatcgctccagggcaaactggaaagattgctgattataattataaattaccagatgattttacaggctgcgttatagcttggaactctaacaatcttgattctaaggttggtggtaattataattacctgtatagattgtttaggaagtctaatctcaaaccttttgagagagatatttcaactgaaatctatcaggccggtagcacaccttgtaatggtgttgaaggttttaattgttactttcctttacaatcatatggtttccaacccactaatggtgttggttaccaaccatacagagtagtagtactttcttttgaacttctacatgcaccagcaactgtttgataagaattctaggctggagcctcggtggccatgcttcttgccccttgggcctccccccagcccctcctccccttcctgcacccgtacccccgtggtctttgaataaagtctgagtgggcggcactagtaaaaaaaaaaaaaaaaaaaaaaaaaaaaaaaaaaaaaaaaaaaaaaaaaaaaaaaaaaaaaaaaaaaaaaaaaaaaaaaaaaaaaaaaaaaaaaaaaaaaaaaaaaaaaaaaaaaaaaaaaaaaaaaaaaaaaaaaaaaaaaaaaaaaaa

SEQ ID NO: 76 - DNA, 1024 bp, synthetic construct
  misc_feature 1..1024: note = mRNA-009 DNA
  source 1..1024: mol_type = other DNA
ggggggatccaagcttagcttgttctttttgcagaagctcagaataaacgctcaactttggcgccgccaccatgtttgtttttcttgttttattgccattagtctctagtagagtccaaccaacagaatctattgttagatttcctaatattacaaacttgtgcccttttggtgaagtttttaacgccaccagatttgcatctgtttatgcttggaacaggaagagaatcagcaactgtgttgctgattattctgtcctatataattccgcatcattttccacttttaagtgttatggagtgtctcctactaaattaaatgatctctgctttactaatgtctatgcagattcatttgtaattagaggtgatgaagtcagacaaatcgctccagggcaaactggaaagattgctgattataattataaattaccagatgattttacaggctgcgttatagcttggaactctaacaatcttgattctaaggttggtggtaattataattacctgtatagattgtttaggaagtctaatctcaaaccttttgagagagatatttcaactgaaatctatcaggccggtagcacaccttgtaatggtgttgaaggttttaattgttactttcctttacaatcatatggtttccaacccactaatggtgttggttaccaaccatacagagtagtagtactttcttttgaacttctacatgcaccagcaactgtttgtggacctaaaaagtgataagaattctaggctggagcctcggtggccatgcttcttgccccttgggcctccccccagcccctcctccccttcctgcacccgtacccccgtggtctttgaataaagtctgagtgggcggcactagtaaaaaaaaaaaaaaaaaaaaaaaaaaaaaaaaaaaaaaaaaaaaaaaaaaaaaaaaaaaaaaaaaaaaaaaaaaaaaaaaaaaaaaaaaaaaaaaaaaaaaaaaaaaaaaaaaaaaaaaaaaaaaaaaaaaaaaaaaaaaaaaaaaaaaa

SEQ ID NO: 77 - RNA, 1025 nt, synthetic construct
  misc_feature 1..1025: note = mRNA-009
  source 1..1025: mol_type = other RNA
gggggggatccaagcttagcttgttctttttgcagaagctcagaataaacgctcaactttggcgccgccaccatgtttgtttttcttgttttattgccattagtctctagtagagtccaaccaacagaatctattgttagatttcctaatattacaaacttgtgcccttttggtgaagtttttaacgccaccagatttgcatctgtttatgcttggaacaggaagagaatcagcaactgtgttgctgattattctgtcctatataattccgcatcattttccacttttaagtgttatggagtgtctcctactaaattaaatgatctctgctttactaatgtctatgcagattcatttgtaattagaggtgatgaagtcagacaaatcgctccagggcaaactggaaagattgctgattataattataaattaccagatgattttacaggctgcgttatagcttggaactctaacaatcttgattctaaggttggtggtaattataattacctgtatagattgtttaggaagtctaatctcaaaccttttgagagagatatttcaactgaaatctatcaggccggtagcacaccttgtaatggtgttgaaggttttaattgttactttcctttacaatcatatggtttccaacccactaatggtgttggttaccaaccatacagagtagtagtactttcttttgaacttctacatgcaccagcaactgtttgtggacctaaaaagtgataagaattctaggctggagcctcggtggccatgcttcttgccccttgggcctccccccagcccctcctccccttcctgcacccgtacccccgtggtctttgaataaagtctgagtgggcggcactagtaaaaaaaaaaaaaaaaaaaaaaaaaaaaaaaaaaaaaaaaaaaaaaaaaaaaaaaaaaaaaaaaaaaaaaaaaaaaaaaaaaaaaaaaaaaaaaaaaaaaaaaaaaaaaaaaaaaaaaaaaaaaaaaaaaaaaaaaaaaaaaaaaaaaaa

SEQ ID NO: 78 - DNA, 1060 bp, synthetic construct
  misc_feature 1..1060: note = mRNA-010 DNA
  source 1..1060: mol_type = other DNA
ggggggatccaagcttagcttgttctttttgcagaagctcagaataaacgctcaactttggcgccgccaccatgtttgtttttcttgttttattgccattagtctctagtagagtccaaccaacagaatctattgttagatttcctaatattacaaacttgtgcccttttggtgaagtttttaacgccaccagatttgcatctgtttatgcttggaacaggaagagaatcagcaactgtgttgctgattattctgtcctatataattccgcatcattttccacttttaagtgttatggagtgtctcctactaaattaaatgatctctgctttactaatgtctatgcagattcatttgtaattagaggtgatgaagtcagacaaatcgctccagggcaaactggaaagattgctgattataattataaattaccagatgattttacaggctgcgttatagcttggaactctaacaatcttgattctaaggttggtggtaattataattacctgtatagattgtttaggaagtctaatctcaaaccttttgagagagatatttcaactgaaatctatcaggccggtagcacaccttgtaatggtgttgaaggttttaattgttactttcctttacaatcatatggtttccaacccactactggtgttggttaccaaccatacagagtagtagtactttcttttgaacttctacatgcaccagcaactgtttgtggacctaaaaagtctactaatttggttaaaaacaaatgtgtcaatttctgataagaattctaggctggagcctcggtggccatgcttcttgccccttgggcctccccccagcccctcctccccttcctgcacccgtacccccgtggtctttgaataaagtctgagtgggcggcactagtaaaaaaaaaaaaaaaaaaaaaaaaaaaaaaaaaaaaaaaaaaaaaaaaaaaaaaaaaaaaaaaaaaaaaaaaaaaaaaaaaaaaaaaaaaaaaaaaaaaaaaaaaaaaaaaaaaaaaaaaaaaaaaaaaaaaaaaaaaaaaaaaaaaaaa

SEQ ID NO: 79 - RNA, 1061 nt, synthetic construct
  misc_feature 1..1061: note = mRNA-010
  source 1..1061: mol_type = other RNA
gggggggatccaagcttagcttgttctttttgcagaagctcagaataaacgctcaactttggcgccgccaccatgtttgtttttcttgttttattgccattagtctctagtagagtccaaccaacagaatctattgttagatttcctaatattacaaacttgtgcccttttggtgaagtttttaacgccaccagatttgcatctgtttatgcttggaacaggaagagaatcagcaactgtgttgctgattattctgtcctatataattccgcatcattttccacttttaagtgttatggagtgtctcctactaaattaaatgatctctgctttactaatgtctatgcagattcatttgtaattagaggtgatgaagtcagacaaatcgctccagggcaaactggaaagattgctgattataattataaattaccagatgattttacaggctgcgttatagcttggaactctaacaatcttgattctaaggttggtggtaattataattacctgtatagattgtttaggaagtctaatctcaaaccttttgagagagatatttcaactgaaatctatcaggccggtagcacaccttgtaatggtgttgaaggttttaattgttactttcctttacaatcatatggtttccaacccactactggtgttggttaccaaccatacagagtagtagtactttcttttgaacttctacatgcaccagcaactgtttgtggacctaaaaagtctactaatttggttaaaaacaaatgtgtcaatttctgataagaattctaggctggagcctcggtggccatgcttcttgccccttgggcctccccccagcccctcctccccttcctgcacccgtacccccgtggtctttgaataaagtctgagtgggcggcactagtaaaaaaaaaaaaaaaaaaaaaaaaaaaaaaaaaaaaaaaaaaaaaaaaaaaaaaaaaaaaaaaaaaaaaaaaaaaaaaaaaaaaaaaaaaaaaaaaaaaaaaaaaaaaaaaaaaaaaaaaaaaaaaaaaaaaaaaaaaaaaaaaaaaaaa

SEQ ID NO: 80 - DNA, 1150 bp, synthetic construct
  misc_feature 1..1150: note = mRNA-011 DNA
  source 1..1150: mol_type = other DNA
ggggggatccaagcttaggcaggagccagggctgggcataaaagtcagggcagagccatctattgcttacatttgcttctgacacaactgtgttcactagcaacctcaaacagacaccgccgccaccatggactggacctggattctcttcttggtggcagcagccacgcgagtccactccagagtccaaccaacagaatctattgttagatttcctaatattacaaacttgtgcccttttggtgaagtttttaacgccaccagatttgcatctgtttatgcttggaacaggaagagaatcagcaactgtgttgctgattattctgtcctatataattccgcatcattttccacttttaagtgttatggagtgtctcctactaaattaaatgatctctgctttactaatgtctatgcagattcatttgtaattagaggtgatgaagtcagacaaatcgctccagggcaaactggaaagattgctgattataattataaattaccagatgattttacaggctgcgttatagcttggaactctaacaatcttgattctaaggttggtggtaattataattacctgtatagattgtttaggaagtctaatctcaaaccttttgagagagatatttcaactgaaatctatcaggccggtagcacaccttgtaatggtgttgaaggttttaattgttactttcctttacaatcatatggtttccaacccactaatggtgttggttaccaaccatacagagtagtagtactttcttttgaacttctacatgcaccagcaactgtttgtggacctaaaaagtctactaatttggttaaaaacaaatgtgtcaatttctgataagaattcgctcgctttcttgctgtccaatttctattaaaggttcctttgttccctaagtccaactactaaactgggggatattatgaagggccttgagcatctggattctgcctaataaaaaacatttattttcattgcactagtaaaaaaaaaaaaaaaaaaaaaaaaaaaaaaaaaaaaaaaaaaaaaaaaaaaaaaaaaaaaaaaaaaaaaaaaaaaaaaaaaaaaaaaaaaaaaaaaaaaaaaaaaaaaaaaaaaaaaaaaaaaaaaaaaaaaaaaaaaaaaaaaaaaaaa

SEQ ID NO: 81 - RNA, 1151 nt, synthetic construct
  misc_feature 1..1151: note = mRNA-011
  source 1..1151: mol_type = other RNA
gggggggatccaagcttaggcaggagccagggctgggcataaaagtcagggcagagccatctattgcttacatttgcttctgacacaactgtgttcactagcaacctcaaacagacaccgccgccaccatggactggacctggattctcttcttggtggcagcagccacgcgagtccactccagagtccaaccaacagaatctattgttagatttcctaatattacaaacttgtgcccttttggtgaagtttttaacgccaccagatttgcatctgtttatgcttggaacaggaagagaatcagcaactgtgttgctgattattctgtcctatataattccgcatcattttccacttttaagtgttatggagtgtctcctactaaattaaatgatctctgctttactaatgtctatgcagattcatttgtaattagaggtgatgaagtcagacaaatcgctccagggcaaactggaaagattgctgattataattataaattaccagatgattttacaggctgcgttatagcttggaactctaacaatcttgattctaaggttggtggtaattataattacctgtatagattgtttaggaagtctaatctcaaaccttttgagagagatatttcaactgaaatctatcaggccggtagcacaccttgtaatggtgttgaaggttttaattgttactttcctttacaatcatatggtttccaacccactaatggtgttggttaccaaccatacagagtagtagtactttcttttgaacttctacatgcaccagcaactgtttgtggacctaaaaagtctactaatttggttaaaaacaaatgtgtcaatttctgataagaattcgctcgctttcttgctgtccaatttctattaaaggttcctttgttccctaagtccaactactaaactgggggatattatgaagggccttgagcatctggattctgcctaataaaaaacatttattttcattgcactagtaaaaaaaaaaaaaaaaaaaaaaaaaaaaaaaaaaaaaaaaaaaaaaaaaaaaaaaaaaaaaaaaaaaaaaaaaaaaaaaaaaaaaaaaaaaaaaaaaaaaaaaaaaaaaaaaaaaaaaaaaaaaaaaaaaaaaaaaaaaaaaaaaaaaaa

SEQ ID NO: 82 - DNA, 1078 bp, synthetic construct
  misc_feature 1..1078: note = mRNA-012 DNA
  source 1..1078: mol_type = other DNA
ggggggatccaagcttaggcaggagccagggctgggcataaaagtcagggcagagccatctattgcttacatttgcttctgacacaactgtgttcactagcaacctcaaacagacaccgccgccaccatggactggacctggattctcttcttggtggcagcagccacgcgagtccactccaatattacaaacttgtgcccttttggtgaagtttttaacgccaccagatttgcatctgtttatgcttggaacaggaagagaatcagcaactgtgttgctgattattctgtcctatataattccgcatcattttccacttttaagtgttatggagtgtctcctactaaattaaatgatctctgctttactaatgtctatgcagattcatttgtaattagaggtgatgaagtcagacaaatcgctccagggcaaactggaaagattgctgattataattataaattaccagatgattttacaggctgcgttatagcttggaactctaacaatcttgattctaaggttggtggtaattataattacctgtatagattgtttaggaagtctaatctcaaaccttttgagagagatatttcaactgaaatctatcaggccggtagcacaccttgtaatggtgttgaaggttttaattgttactttcctttacaatcatatggtttccaacccactaatggtgttggttaccaaccatacagagtagtagtactttcttttgaacttctacatgcaccagcaactgtttgtggacctaaaaagtgataagaattcgctcgctttcttgctgtccaatttctattaaaggttcctttgttccctaagtccaactactaaactgggggatattatgaagggccttgagcatctggattctgcctaataaaaaacatttattttcattgcactagtaaaaaaaaaaaaaaaaaaaaaaaaaaaaaaaaaaaaaaaaaaaaaaaaaaaaaaaaaaaaaaaaaaaaaaaaaaaaaaaaaaaaaaaaaaaaaaaaaaaaaaaaaaaaaaaaaaaaaaaaaaaaaaaaaaaaaaaaaaaaaaaaaaaaaa

SEQ ID NO: 83 - RNA, 1079 nt, synthetic construct
  misc_feature 1..1079: note = mRNA-012
  source 1..1079: mol_type = other RNA
gggggggatccaagcttaggcaggagccagggctgggcataaaagtcagggcagagccatctattgcttacatttgcttctgacacaactgtgttcactagcaacctcaaacagacaccgccgccaccatggactggacctggattctcttcttggtggcagcagccacgcgagtccactccaatattacaaacttgtgcccttttggtgaagtttttaacgccaccagatttgcatctgtttatgcttggaacaggaagagaatcagcaactgtgttgctgattattctgtcctatataattccgcatcattttccacttttaagtgttatggagtgtctcctactaaattaaatgatctctgctttactaatgtctatgcagattcatttgtaattagaggtgatgaagtcagacaaatcgctccagggcaaactggaaagattgctgattataattataaattaccagatgattttacaggctgcgttatagcttggaactctaacaatcttgattctaaggttggtggtaattataattacctgtatagattgtttaggaagtctaatctcaaaccttttgagagagatatttcaactgaaatctatcaggccggtagcacaccttgtaatggtgttgaaggttttaattgttactttcctttacaatcatatggtttccaacccactaatggtgttggttaccaaccatacagagtagtagtactttcttttgaacttctacatgcaccagcaactgtttgtggacctaaaaagtgataagaattcgctcgctttcttgctgtccaatttctattaaaggttcctttgttccctaagtccaactactaaactgggggatattatgaagggccttgagcatctggattctgcctaataaaaaacatttattttcattgcactagtaaaaaaaaaaaaaaaaaaaaaaaaaaaaaaaaaaaaaaaaaaaaaaaaaaaaaaaaaaaaaaaaaaaaaaaaaaaaaaaaaaaaaaaaaaaaaaaaaaaaaaaaaaaaaaaaaaaaaaaaaaaaaaaaaaaaaaaaaaaaaaaaaaaaaa

SEQ ID NO: 84 - DNA, 1063 bp, synthetic construct
  misc_feature 1..1063: note = mRNA-013 DNA
  source 1..1063: mol_type = other DNA
ggggggatccaagcttaggcaggagccagggctgggcataaaagtcagggcagagccatctattgcttacatttgcttctgacacaactgtgttcactagcaacctcaaacagacaccgccgccaccatggactggacctggattctcttcttggtggcagcagccacgcgagtccactccaatattacaaacttgtgcccttttggtgaagtttttaacgccaccagatttgcatctgtttatgcttggaacaggaagagaatcagcaactgtgttgctgattattctgtcctatataattccgcatcattttccacttttaagtgttatggagtgtctcctactaaattaaatgatctctgctttactaatgtctatgcagattcatttgtaattagaggtgatgaagtcagacaaatcgctccagggcaaactggaaagattgctgattataattataaattaccagatgattttacaggctgcgttatagcttggaactctaacaatcttgattctaaggttggtggtaattataattacctgtatagattgtttaggaagtctaatctcaaaccttttgagagagatatttcaactgaaatctatcaggccggtagcacaccttgtaatggtgttgaaggttttaattgttactttcctttacaatcatatggtttccaacccactaatggtgttggttaccaaccatacagagtagtagtactttcttttgaacttctacatgcaccagcaactgtttgataagaattcgctcgctttcttgctgtccaatttctattaaaggttcctttgttccctaagtccaactactaaactgggggatattatgaagggccttgagcatctggattctgcctaataaaaaacatttattttcattgcactagtaaaaaaaaaaaaaaaaaaaaaaaaaaaaaaaaaaaaaaaaaaaaaaaaaaaaaaaaaaaaaaaaaaaaaaaaaaaaaaaaaaaaaaaaaaaaaaaaaaaaaaaaaaaaaaaaaaaaaaaaaaaaaaaaaaaaaaaaaaaaaaaaaaaaaa

SEQ ID NO: 85 - RNA, 1064 nt, synthetic construct
  misc_feature 1..1064: note = mRNA-013
  source 1..1064: mol_type = other RNA
gggggggatccaagcttaggcaggagccagggctgggcataaaagtcagggcagagccatctattgcttacatttgcttctgacacaactgtgttcactagcaacctcaaacagacaccgccgccaccatggactggacctggattctcttcttggtggcagcagccacgcgagtccactccaatattacaaacttgtgcccttttggtgaagtttttaacgccaccagatttgcatctgtttatgcttggaacaggaagagaatcagcaactgtgttgctgattattctgtcctatataattccgcatcattttccacttttaagtgttatggagtgtctcctactaaattaaatgatctctgctttactaatgtctatgcagattcatttgtaattagaggtgatgaagtcagacaaatcgctccagggcaaactggaaagattgctgattataattataaattaccagatgattttacaggctgcgttatagcttggaactctaacaatcttgattctaaggttggtggtaattataattacctgtatagattgtttaggaagtctaatctcaaaccttttgagagagatatttcaactgaaatctatcaggccggtagcacaccttgtaatggtgttgaaggttttaattgttactttcctttacaatcatatggtttccaacccactaatggtgttggttaccaaccatacagagtagtagtactttcttttgaacttctacatgcaccagcaactgtttgataagaattcgctcgctttcttgctgtccaatttctattaaaggttcctttgttccctaagtccaactactaaactgggggatattatgaagggccttgagcatctggattctgcctaataaaaaacatttattttcattgcactagtaaaaaaaaaaaaaaaaaaaaaaaaaaaaaaaaaaaaaaaaaaaaaaaaaaaaaaaaaaaaaaaaaaaaaaaaaaaaaaaaaaaaaaaaaaaaaaaaaaaaaaaaaaaaaaaaaaaaaaaaaaaaaaaaaaaaaaaaaaaaaaaaaaaaaa

SEQ ID NO: 86 - DNA, 1114 bp, synthetic construct
  misc_feature 1..1114: note = mRNA-014 DNA
  source 1..1114: mol_type = other DNA
ggggggatccaagcttaggcaggagccagggctgggcataaaagtcagggcagagccatctattgcttacatttgcttctgacacaactgtgttcactagcaacctcaaacagacaccgccgccaccatggactggacctggattctcttcttggtggcagcagccacgcgagtccactccagagtccaaccaacagaatctattgttagatttcctaatattacaaacttgtgcccttttggtgaagtttttaacgccaccagatttgcatctgtttatgcttggaacaggaagagaatcagcaactgtgttgctgattattctgtcctatataattccgcatcattttccacttttaagtgttatggagtgtctcctactaaattaaatgatctctgctttactaatgtctatgcagattcatttgtaattagaggtgatgaagtcagacaaatcgctccagggcaaactggaaagattgctgattataattataaattaccagatgattttacaggctgcgttatagcttggaactctaacaatcttgattctaaggttggtggtaattataattacctgtatagattgtttaggaagtctaatctcaaaccttttgagagagatatttcaactgaaatctatcaggccggtagcacaccttgtaatggtgttgaaggttttaattgttactttcctttacaatcatatggtttccaacccactaatggtgttggttaccaaccatacagagtagtagtactttcttttgaacttctacatgcaccagcaactgtttgtggacctaaaaagtgataagaattcgctcgctttcttgctgtccaatttctattaaaggttcctttgttccctaagtccaactactaaactgggggatattatgaagggccttgagcatctggattctgcctaataaaaaacatttattttcattgcactagtaaaaaaaaaaaaaaaaaaaaaaaaaaaaaaaaaaaaaaaaaaaaaaaaaaaaaaaaaaaaaaaaaaaaaaaaaaaaaaaaaaaaaaaaaaaaaaaaaaaaaaaaaaaaaaaaaaaaaaaaaaaaaaaaaaaaaaaaaaaaaaaaaaaaaa

SEQ ID NO: 87 - RNA, 1115 nt, synthetic construct
  misc_feature 1..1115: note = mRNA-014
  source 1..1115: mol_type = other RNA
gggggggatccaagcttaggcaggagccagggctgggcataaaagtcagggcagagccatctattgcttacatttgcttctgacacaactgtgttcactagcaacctcaaacagacaccgccgccaccatggactggacctggattctcttcttggtggcagcagccacgcgagtccactccagagtccaaccaacagaatctattgttagatttcctaatattacaaacttgtgcccttttggtgaagtttttaacgccaccagatttgcatctgtttatgcttggaacaggaagagaatcagcaactgtgttgctgattattctgtcctatataattccgcatcattttccacttttaagtgttatggagtgtctcctactaaattaaatgatctctgctttactaatgtctatgcagattcatttgtaattagaggtgatgaagtcagacaaatcgctccagggcaaactggaaagattgctgattataattataaattaccagatgattttacaggctgcgttatagcttggaactctaacaatcttgattctaaggttggtggtaattataattacctgtatagattgtttaggaagtctaatctcaaaccttttgagagagatatttcaactgaaatctatcaggccggtagcacaccttgtaatggtgttgaaggttttaattgttactttcctttacaatcatatggtttccaacccactaatggtgttggttaccaaccatacagagtagtagtactttcttttgaacttctacatgcaccagcaactgtttgtggacctaaaaagtgataagaattcgctcgctttcttgctgtccaatttctattaaaggttcctttgttccctaagtccaactactaaactgggggatattatgaagggccttgagcatctggattctgcctaataaaaaacatttattttcattgcactagtaaaaaaaaaaaaaaaaaaaaaaaaaaaaaaaaaaaaaaaaaaaaaaaaaaaaaaaaaaaaaaaaaaaaaaaaaaaaaaaaaaaaaaaaaaaaaaaaaaaaaaaaaaaaaaaaaaaaaaaaaaaaaaaaaaaaaaaaaaaaaaaaaaaaaa

SEQ ID NO: 88 - DNA, 1150 bp, synthetic construct
  misc_feature 1..1150: note = mRNA-015 DNA
  source 1..1150: mol_type = other DNA
ggggggatccaagcttaggcaggagccagggctgggcataaaagtcagggcagagccatctattgcttacatttgcttctgacacaactgtgttcactagcaacctcaaacagacaccgccgccaccatggactggacctggattctcttcttggtggcagcagccacgcgagtccactccagagtccaaccaacagaatctattgttagatttcctaatattacaaacttgtgcccttttggtgaagtttttaacgccaccagatttgcatctgtttatgcttggaacaggaagagaatcagcaactgtgttgctgattattctgtcctatataattccgcatcattttccacttttaagtgttatggagtgtctcctactaaattaaatgatctctgctttactaatgtctatgcagattcatttgtaattagaggtgatgaagtcagacaaatcgctccagggcaaactggaaagattgctgattataattataaattaccagatgattttacaggctgcgttatagcttggaactctaacaatcttgattctaaggttggtggtaattataattacctgtatagattgtttaggaagtctaatctcaaaccttttgagagagatatttcaactgaaatctatcaggccggtagcacaccttgtaatggtgttgaaggttttaattgttactttcctttacaatcatatggtttccaacccactactggtgttggttaccaaccatacagagtagtagtactttcttttgaacttctacatgcaccagcaactgtttgtggacctaaaaagtctactaatttggttaaaaacaaatgtgtcaatttctgataagaattcgctcgctttcttgctgtccaatttctattaaaggttcctttgttccctaagtccaactactaaactgggggatattatgaagggccttgagcatctggattctgcctaataaaaaacatttattttcattgcactagtaaaaaaaaaaaaaaaaaaaaaaaaaaaaaaaaaaaaaaaaaaaaaaaaaaaaaaaaaaaaaaaaaaaaaaaaaaaaaaaaaaaaaaaaaaaaaaaaaaaaaaaaaaaaaaaaaaaaaaaaaaaaaaaaaaaaaaaaaaaaaaaaaaaaaa

SEQ ID NO: 89 - RNA, 1151 nt, synthetic construct
  misc_feature 1..1151: note = mRNA-015
  source 1..1151: mol_type = other RNA
gggggggatccaagcttaggcaggagccagggctgggcataaaagtcagggcagagccatctattgcttacatttgcttctgacacaactgtgttcactagcaacctcaaacagacaccgccgccaccatggactggacctggattctcttcttggtggcagcagccacgcgagtccactccagagtccaaccaacagaatctattgttagatttcctaatattacaaacttgtgcccttttggtgaagtttttaacgccaccagatttgcatctgtttatgcttggaacaggaagagaatcagcaactgtgttgctgattattctgtcctatataattccgcatcattttccacttttaagtgttatggagtgtctcctactaaattaaatgatctctgctttactaatgtctatgcagattcatttgtaattagaggtgatgaagtcagacaaatcgctccagggcaaactggaaagattgctgattataattataaattaccagatgattttacaggctgcgttatagcttggaactctaacaatcttgattctaaggttggtggtaattataattacctgtatagattgtttaggaagtctaatctcaaaccttttgagagagatatttcaactgaaatctatcaggccggtagcacaccttgtaatggtgttgaaggttttaattgttactttcctttacaatcatatggtttccaacccactactggtgttggttaccaaccatacagagtagtagtactttcttttgaacttctacatgcaccagcaactgtttgtggacctaaaaagtctactaatttggttaaaaacaaatgtgtcaatttctgataagaattcgctcgctttcttgctgtccaatttctattaaaggttcctttgttccctaagtccaactactaaactgggggatattatgaagggccttgagcatctggattctgcctaataaaaaacatttattttcattgcactagtaaaaaaaaaaaaaaaaaaaaaaaaaaaaaaaaaaaaaaaaaaaaaaaaaaaaaaaaaaaaaaaaaaaaaaaaaaaaaaaaaaaaaaaaaaaaaaaaaaaaaaaaaaaaaaaaaaaaaaaaaaaaaaaaaaaaaaaaaaaaaaaaaaaaaa

SEQ ID NO: 90 - DNA, 1135 bp, synthetic construct
  misc_feature 1..1135: note = mRNA-016 DNA
  source 1..1135: mol_type = other DNA
ggggggatccaagcttaggcaggagccagggctgggcataaaagtcagggcagagccatctattgcttacatttgcttctgacacaactgtgttcactagcaacctcaaacagacaccgccgccaccatgtttgtttttcttgttttattgccattagtctctagtagagtccaaccaacagaatctattgttagatttcctaatattacaaacttgtgcccttttggtgaagtttttaacgccaccagatttgcatctgtttatgcttggaacaggaagagaatcagcaactgtgttgctgattattctgtcctatataattccgcatcattttccacttttaagtgttatggagtgtctcctactaaattaaatgatctctgctttactaatgtctatgcagattcatttgtaattagaggtgatgaagtcagacaaatcgctccagggcaaactggaaagattgctgattataattataaattaccagatgattttacaggctgcgttatagcttggaactctaacaatcttgattctaaggttggtggtaattataattacctgtatagattgtttaggaagtctaatctcaaaccttttgagagagatatttcaactgaaatctatcaggccggtagcacaccttgtaatggtgttgaaggttttaattgttactttcctttacaatcatatggtttccaacccactaatggtgttggttaccaaccatacagagtagtagtactttcttttgaacttctacatgcaccagcaactgtttgtggacctaaaaagtctactaatttggttaaaaacaaatgtgtcaatttctgataagaattcgctcgctttcttgctgtccaatttctattaaaggttcctttgttccctaagtccaactactaaactgggggatattatgaagggccttgagcatctggattctgcctaataaaaaacatttattttcattgcactagtaaaaaaaaaaaaaaaaaaaaaaaaaaaaaaaaaaaaaaaaaaaaaaaaaaaaaaaaaaaaaaaaaaaaaaaaaaaaaaaaaaaaaaaaaaaaaaaaaaaaaaaaaaaaaaaaaaaaaaaaaaaaaaaaaaaaaaaaaaaaaaaaaaaaaa

SEQ ID NO: 91 - RNA, 1136 nt, synthetic construct
  misc_feature 1..1136: note = mRNA-016
  source 1..1136: mol_type = other RNA
gggggggatccaagcttaggcaggagccagggctgggcataaaagtcagggcagagccatctattgcttacatttgcttctgacacaactgtgttcactagcaacctcaaacagacaccgccgccaccatgtttgtttttcttgttttattgccattagtctctagtagagtccaaccaacagaatctattgttagatttcctaatattacaaacttgtgcccttttggtgaagtttttaacgccaccagatttgcatctgtttatgcttggaacaggaagagaatcagcaactgtgttgctgattattctgtcctatataattccgcatcattttccacttttaagtgttatggagtgtctcctactaaattaaatgatctctgctttactaatgtctatgcagattcatttgtaattagaggtgatgaagtcagacaaatcgctccagggcaaactggaaagattgctgattataattataaattaccagatgattttacaggctgcgttatagcttggaactctaacaatcttgattctaaggttggtggtaattataattacctgtatagattgtttaggaagtctaatctcaaaccttttgagagagatatttcaactgaaatctatcaggccggtagcacaccttgtaatggtgttgaaggttttaattgttactttcctttacaatcatatggtttccaacccactaatggtgttggttaccaaccatacagagtagtagtactttcttttgaacttctacatgcaccagcaactgtttgtggacctaaaaagtctactaatttggttaaaaacaaatgtgtcaatttctgataagaattcgctcgctttcttgctgtccaatttctattaaaggttcctttgttccctaagtccaactactaaactgggggatattatgaagggccttgagcatctggattctgcctaataaaaaacatttattttcattgcactagtaaaaaaaaaaaaaaaaaaaaaaaaaaaaaaaaaaaaaaaaaaaaaaaaaaaaaaaaaaaaaaaaaaaaaaaaaaaaaaaaaaaaaaaaaaaaaaaaaaaaaaaaaaaaaaaaaaaaaaaaaaaaaaaaaaaaaaaaaaaaaaaaaaaaaa

SEQ ID NO: 92 - DNA, 1063 bp, synthetic construct
  misc_feature 1..1063: note = mRNA-017 DNA
  source 1..1063: mol_type = other DNA
ggggggatccaagcttaggcaggagccagggctgggcataaaagtcagggcagagccatctattgcttacatttgcttctgacacaactgtgttcactagcaacctcaaacagacaccgccgccaccatgtttgtttttcttgttttattgccattagtctctagtaatattacaaacttgtgcccttttggtgaagtttttaacgccaccagatttgcatctgtttatgcttggaacaggaagagaatcagcaactgtgttgctgattattctgtcctatataattccgcatcattttccacttttaagtgttatggagtgtctcctactaaattaaatgatctctgctttactaatgtctatgcagattcatttgtaattagaggtgatgaagtcagacaaatcgctccagggcaaactggaaagattgctgattataattataaattaccagatgattttacaggctgcgttatagcttggaactctaacaatcttgattctaaggttggtggtaattataattacctgtatagattgtttaggaagtctaatctcaaaccttttgagagagatatttcaactgaaatctatcaggccggtagcacaccttgtaatggtgttgaaggttttaattgttactttcctttacaatcatatggtttccaacccactaatggtgttggttaccaaccatacagagtagtagtactttcttttgaacttctacatgcaccagcaactgtttgtggacctaaaaagtgataagaattcgctcgctttcttgctgtccaatttctattaaaggttcctttgttccctaagtccaactactaaactgggggatattatgaagggccttgagcatctggattctgcctaataaaaaacatttattttcattgcactagtaaaaaaaaaaaaaaaaaaaaaaaaaaaaaaaaaaaaaaaaaaaaaaaaaaaaaaaaaaaaaaaaaaaaaaaaaaaaaaaaaaaaaaaaaaaaaaaaaaaaaaaaaaaaaaaaaaaaaaaaaaaaaaaaaaaaaaaaaaaaaaaaaaaaaa

SEQ ID NO: 93 - RNA, 1064 nt, synthetic construct
  misc_feature 1..1064: note = mRNA-017
  source 1..1064: mol_type = other RNA
gggggggatccaagcttaggcaggagccagggctgggcataaaagtcagggcagagccatctattgcttacatttgcttctgacacaactgtgttcactagcaacctcaaacagacaccgccgccaccatgtttgtttttcttgttttattgccattagtctctagtaatattacaaacttgtgcccttttggtgaagtttttaacgccaccagatttgcatctgtttatgcttggaacaggaagagaatcagcaactgtgttgctgattattctgtcctatataattccgcatcattttccacttttaagtgttatggagtgtctcctactaaattaaatgatctctgctttactaatgtctatgcagattcatttgtaattagaggtgatgaagtcagacaaatcgctccagggcaaactggaaagattgctgattataattataaattaccagatgattttacaggctgcgttatagcttggaactctaacaatcttgattctaaggttggtggtaattataattacctgtatagattgtttaggaagtctaatctcaaaccttttgagagagatatttcaactgaaatctatcaggccggtagcacaccttgtaatggtgttgaaggttttaattgttactttcctttacaatcatatggtttccaacccactaatggtgttggttaccaaccatacagagtagtagtactttcttttgaacttctacatgcaccagcaactgtttgtggacctaaaaagtgataagaattcgctcgctttcttgctgtccaatttctattaaaggttcctttgttccctaagtccaactactaaactgggggatattatgaagggccttgagcatctggattctgcctaataaaaaacatttattttcattgcactagtaaaaaaaaaaaaaaaaaaaaaaaaaaaaaaaaaaaaaaaaaaaaaaaaaaaaaaaaaaaaaaaaaaaaaaaaaaaaaaaaaaaaaaaaaaaaaaaaaaaaaaaaaaaaaaaaaaaaaaaaaaaaaaaaaaaaaaaaaaaaaaaaaaaaaa

SEQ ID NO: 94 - DNA, 1048 bp, synthetic construct
  misc_feature 1..1048: note = mRNA-018 DNA
  source 1..1048: mol_type = other DNA
ggggggatccaagcttaggcaggagccagggctgggcataaaagtcagggcagagccatctattgcttacatttgcttctgacacaactgtgttcactagcaacctcaaacagacaccgccgccaccatgtttgtttttcttgttttattgccattagtctctagtaatattacaaacttgtgcccttttggtgaagtttttaacgccaccagatttgcatctgtttatgcttggaacaggaagagaatcagcaactgtgttgctgattattctgtcctatataattccgcatcattttccacttttaagtgttatggagtgtctcctactaaattaaatgatctctgctttactaatgtctatgcagattcatttgtaattagaggtgatgaagtcagacaaatcgctccagggcaaactggaaagattgctgattataattataaattaccagatgattttacaggctgcgttatagcttggaactctaacaatcttgattctaaggttggtggtaattataattacctgtatagattgtttaggaagtctaatctcaaaccttttgagagagatatttcaactgaaatctatcaggccggtagcacaccttgtaatggtgttgaaggttttaattgttactttcctttacaatcatatggtttccaacccactaatggtgttggttaccaaccatacagagtagtagtactttcttttgaacttctacatgcaccagcaactgtttgataagaattcgctcgctttcttgctgtccaatttctattaaaggttcctttgttccctaagtccaactactaaactgggggatattatgaagggccttgagcatctggattctgcctaataaaaaacatttattttcattgcactagtaaaaaaaaaaaaaaaaaaaaaaaaaaaaaaaaaaaaaaaaaaaaaaaaaaaaaaaaaaaaaaaaaaaaaaaaaaaaaaaaaaaaaaaaaaaaaaaaaaaaaaaaaaaaaaaaaaaaaaaaaaaaaaaaaaaaaaaaaaaaaaaaaaaaaa

SEQ ID NO: 95 - RNA, 1049 nt, synthetic construct
  misc_feature 1..1049: note = mRNA-018
  source 1..1049: mol_type = other RNA
gggggggatccaagcttaggcaggagccagggctgggcataaaagtcagggcagagccatctattgcttacatttgcttctgacacaactgtgttcactagcaacctcaaacagacaccgccgccaccatgtttgtttttcttgttttattgccattagtctctagtaatattacaaacttgtgcccttttggtgaagtttttaacgccaccagatttgcatctgtttatgcttggaacaggaagagaatcagcaactgtgttgctgattattctgtcctatataattccgcatcattttccacttttaagtgttatggagtgtctcctactaaattaaatgatctctgctttactaatgtctatgcagattcatttgtaattagaggtgatgaagtcagacaaatcgctccagggcaaactggaaagattgctgattataattataaattaccagatgattttacaggctgcgttatagcttggaactctaacaatcttgattctaaggttggtggtaattataattacctgtatagattgtttaggaagtctaatctcaaaccttttgagagagatatttcaactgaaatctatcaggccggtagcacaccttgtaatggtgttgaaggttttaattgttactttcctttacaatcatatggtttccaacccactaatggtgttggttaccaaccatacagagtagtagtactttcttttgaacttctacatgcaccagcaactgtttgataagaattcgctcgctttcttgctgtccaatttctattaaaggttcctttgttccctaagtccaactactaaactgggggatattatgaagggccttgagcatctggattctgcctaataaaaaacatttattttcattgcactagtaaaaaaaaaaaaaaaaaaaaaaaaaaaaaaaaaaaaaaaaaaaaaaaaaaaaaaaaaaaaaaaaaaaaaaaaaaaaaaaaaaaaaaaaaaaaaaaaaaaaaaaaaaaaaaaaaaaaaaaaaaaaaaaaaaaaaaaaaaaaaaaaaaaaaa

SEQ ID NO: 96 - DNA, 1099 bp, synthetic construct
  misc_feature 1..1099: note = mRNA-019 DNA
  source 1..1099: mol_type = other DNA
ggggggatccaagcttaggcaggagccagggctgggcataaaagtcagggcagagccatctattgcttacatttgcttctgacacaactgtgttcactagcaacctcaaacagacaccgccgccaccatgtttgtttttcttgttttattgccattagtctctagtagagtccaaccaacagaatctattgttagatttcctaatattacaaacttgtgcccttttggtgaagtttttaacgccaccagatttgcatctgtttatgcttggaacaggaagagaatcagcaactgtgttgctgattattctgtcctatataattccgcatcattttccacttttaagtgttatggagtgtctcctactaaattaaatgatctctgctttactaatgtctatgcagattcatttgtaattagaggtgatgaagtcagacaaatcgctccagggcaaactggaaagattgctgattataattataaattaccagatgattttacaggctgcgttatagcttggaactctaacaatcttgattctaaggttggtggtaattataattacctgtatagattgtttaggaagtctaatctcaaaccttttgagagagatatttcaactgaaatctatcaggccggtagcacaccttgtaatggtgttgaaggttttaattgttactttcctttacaatcatatggtttccaacccactaatggtgttggttaccaaccatacagagtagtagtactttcttttgaacttctacatgcaccagcaactgtttgtggacctaaaaagtgataagaattcgctcgctttcttgctgtccaatttctattaaaggttcctttgttccctaagtccaactactaaactgggggatattatgaagggccttgagcatctggattctgcctaataaaaaacatttattttcattgcactagtaaaaaaaaaaaaaaaaaaaaaaaaaaaaaaaaaaaaaaaaaaaaaaaaaaaaaaaaaaaaaaaaaaaaaaaaaaaaaaaaaaaaaaaaaaaaaaaaaaaaaaaaaaaaaaaaaaaaaaaaaaaaaaaaaaaaaaaaaaaaaaaaaaaaaa

SEQ ID NO: 97 - RNA, 1100 nt, synthetic construct
  misc_feature 1..1100: note = mRNA-019
  source 1..1100: mol_type = other RNA
gggggggatccaagcttaggcaggagccagggctgggcataaaagtcagggcagagccatctattgcttacatttgcttctgacacaactgtgttcactagcaacctcaaacagacaccgccgccaccatgtttgtttttcttgttttattgccattagtctctagtagagtccaaccaacagaatctattgttagatttcctaatattacaaacttgtgcccttttggtgaagtttttaacgccaccagatttgcatctgtttatgcttggaacaggaagagaatcagcaactgtgttgctgattattctgtcctatataattccgcatcattttccacttttaagtgttatggagtgtctcctactaaattaaatgatctctgctttactaatgtctatgcagattcatttgtaattagaggtgatgaagtcagacaaatcgctccagggcaaactggaaagattgctgattataattataaattaccagatgattttacaggctgcgttatagcttggaactctaacaatcttgattctaaggttggtggtaattataattacctgtatagattgtttaggaagtctaatctcaaaccttttgagagagatatttcaactgaaatctatcaggccggtagcacaccttgtaatggtgttgaaggttttaattgttactttcctttacaatcatatggtttccaacccactaatggtgttggttaccaaccatacagagtagtagtactttcttttgaacttctacatgcaccagcaactgtttgtggacctaaaaagtgataagaattcgctcgctttcttgctgtccaatttctattaaaggttcctttgttccctaagtccaactactaaactgggggatattatgaagggccttgagcatctggattctgcctaataaaaaacatttattttcattgcactagtaaaaaaaaaaaaaaaaaaaaaaaaaaaaaaaaaaaaaaaaaaaaaaaaaaaaaaaaaaaaaaaaaaaaaaaaaaaaaaaaaaaaaaaaaaaaaaaaaaaaaaaaaaaaaaaaaaaaaaaaaaaaaaaaaaaaaaaaaaaaaaaaaaaaaa

SEQ ID NO: 98 - DNA, 1135 bp, synthetic construct
  misc_feature 1..1135: note = mRNA-020 DNA
  source 1..1135: mol_type = other DNA
ggggggatccaagcttaggcaggagccagggctgggcataaaagtcagggcagagccatctattgcttacatttgcttctgacacaactgtgttcactagcaacctcaaacagacaccgccgccaccatgtttgtttttcttgttttattgccattagtctctagtagagtccaaccaacagaatctattgttagatttcctaatattacaaacttgtgcccttttggtgaagtttttaacgccaccagatttgcatctgtttatgcttggaacaggaagagaatcagcaactgtgttgctgattattctgtcctatataattccgcatcattttccacttttaagtgttatggagtgtctcctactaaattaaatgatctctgctttactaatgtctatgcagattcatttgtaattagaggtgatgaagtcagacaaatcgctccagggcaaactggaaagattgctgattataattataaattaccagatgattttacaggctgcgttatagcttggaactctaacaatcttgattctaaggttggtggtaattataattacctgtatagattgtttaggaagtctaatctcaaaccttttgagagagatatttcaactgaaatctatcaggccggtagcacaccttgtaatggtgttgaaggttttaattgttactttcctttacaatcatatggtttccaacccactactggtgttggttaccaaccatacagagtagtagtactttcttttgaacttctacatgcaccagcaactgtttgtggacctaaaaagtctactaatttggttaaaaacaaatgtgtcaatttctgataagaattcgctcgctttcttgctgtccaatttctattaaaggttcctttgttccctaagtccaactactaaactgggggatattatgaagggccttgagcatctggattctgcctaataaaaaacatttattttcattgcactagtaaaaaaaaaaaaaaaaaaaaaaaaaaaaaaaaaaaaaaaaaaaaaaaaaaaaaaaaaaaaaaaaaaaaaaaaaaaaaaaaaaaaaaaaaaaaaaaaaaaaaaaaaaaaaaaaaaaaaaaaaaaaaaaaaaaaaaaaaaaaaaaaaaaaaa

SEQ ID NO: 99 - RNA, 1136 nt, synthetic construct
  misc_feature 1..1136: note = mRNA-020
  source 1..1136: mol_type = other RNA
gggggggatccaagcttaggcaggagccagggctgggcataaaagtcagggcagagccatctattgcttacatttgcttctgacacaactgtgttcactagcaacctcaaacagacaccgccgccaccatgtttgtttttcttgttttattgccattagtctctagtagagtccaaccaacagaatctattgttagatttcctaatattacaaacttgtgcccttttggtgaagtttttaacgccaccagatttgcatctgtttatgcttggaacaggaagagaatcagcaactgtgttgctgattattctgtcctatataattccgcatcattttccacttttaagtgttatggagtgtctcctactaaattaaatgatctctgctttactaatgtctatgcagattcatttgtaattagaggtgatgaagtcagacaaatcgctccagggcaaactggaaagattgctgattataattataaattaccagatgattttacaggctgcgttatagcttggaactctaacaatcttgattctaaggttggtggtaattataattacctgtatagattgtttaggaagtctaatctcaaaccttttgagagagatatttcaactgaaatctatcaggccggtagcacaccttgtaatggtgttgaaggttttaattgttactttcctttacaatcatatggtttccaacccactactggtgttggttaccaaccatacagagtagtagtactttcttttgaacttctacatgcaccagcaactgtttgtggacctaaaaagtctactaatttggttaaaaacaaatgtgtcaatttctgataagaattcgctcgctttcttgctgtccaatttctattaaaggttcctttgttccctaagtccaactactaaactgggggatattatgaagggccttgagcatctggattctgcctaataaaaaacatttattttcattgcactagtaaaaaaaaaaaaaaaaaaaaaaaaaaaaaaaaaaaaaaaaaaaaaaaaaaaaaaaaaaaaaaaaaaaaaaaaaaaaaaaaaaaaaaaaaaaaaaaaaaaaaaaaaaaaaaaaaaaaaaaaaaaaaaaaaaaaaaaaaaaaaaaaaaaaaa